European Patent Application EP 4 234 581 A2, published August 30, 2023. Title: Therapeutic antibodies and their uses. Applicant: Pfizer Inc. Application EP. The sequence listing filed with the application follows.

SEQUENCE LISTING (502 sequences)

SEQ ID NO: 1 - protein, 109 aa, synthetic construct
  REGION 1..109: note = Synthetic Construct
EIVLTQSPGTLSLSPGERATLSCRASQSVSSSYLAWYQQKPGQAPRLLIYGASSRATGIPDRFSGSGSGTDFTLTISRLEPEDFAVYYCQHYGSPPSFTFGQGTKVEIK

SEQ ID NO: 2 - protein, 119 aa, synthetic construct
  REGION 1..119: note = Synthetic Construct
EVQLLESGGGLVQPGGSLRLSCAASGFTFGSYAMTWVRQAPGKGLEWVSAISGSGGNTFYADSVKGRFTISRDNSKNTLYLQMNSLRAEDTAVYYCARVSPIASGMDYWGQGTLVTVSS

SEQ ID NO: 3 - protein, 119 aa, synthetic construct
  REGION 1..119: note = Synthetic Construct
EVQLLESGGGLVQPGGSLRLSCAASGFTFGSYAMTWVRQAPGKGLEWVSAISGSGGNTFYADSVKGRFTISRDNSKNTLYLQMNSLRAEDTAVYYCARVSPIAAQMDYWGQGTLVTVSS

SEQ ID NO: 4 - protein, 109 aa, synthetic construct
  REGION 1..109: note = Synthetic Construct
EIVLTQSPGTLSLSPGERATLSCRASQSLGSFYLAWYQQKPGQAPRLLIYGASSRATGIPDRFSGSGSGTDFTLTISRLEPEDFAVYYCKHYGWPPSFTFGQGTKVEIK

SEQ ID NO: 5 - protein, 109 aa, synthetic construct
  REGION 1..109: note = Synthetic Construct
EIVLTQSPGTLSLSPGERATLSCRASQSLGSFYLAWYQQKPGQAPRLLIYGASSRATGIPDRFSGSGSGTDFTLTISRLEPEDFAVYYCQHYNYPPSFTFGQGTKVEIK

SEQ ID NO: 6 - protein, 109 aa, synthetic construct
  REGION 1..109: note = Synthetic Construct
EIVLTQSPGTLSLSPGERATLSCRASQSVGDFYLAWYQQKPGQAPRLLIYGASSRATGIPDRFSGSGSGTDFTLTISRLEPEDFAVYYCQHYNYPPSFTFGQGTKVEIK

SEQ ID NO: 7 - protein, 121 aa, synthetic construct
  REGION 1..121: note = Synthetic Construct
EVQLLESGGGLVQPGGSLRLSCAASGFTFGSYAMTWVRQAPGKGLEWVSAISGSGGNTFYADSVKGRFTISRDNSKNTLYLQMNSLRAEDTAVYYCARARVSPIAALMDYWGQGTLVTVSS

SEQ ID NO: 8 - protein, 119 aa, synthetic construct
  REGION 1..119: note = Synthetic Construct
EVQLLESGGGLVQPGGSLRLSCAASGFTFGSYAMTWVRQAPGKGLEWVSAISGSGGNTFYADSVKGRFTISRDNSKNTLYLQMNSLRAEDTAVYYCARVSPIAAPMDYWGQGTLVTVSS

SEQ ID NO: 9 - protein, 109 aa, synthetic construct
  REGION 1..109: note = Synthetic Construct
EIVLTQSPGTLSLSPGERATLSCRASQSLGSFYLAWYQQKPGQAPRLLIYGASSRATGIPDRFSGSGSGTDFTLTISRLEPEDFAVYYCQHYPYPPSFTFGQGTKVEIK

SEQ ID NO: 10 - protein, 109 aa, synthetic construct; identical to SEQ ID NO: 5
  REGION 1..109: note = Synthetic Construct

SEQ ID NO: 11 - protein, 109 aa, synthetic construct
  REGION 1..109: note = Synthetic Construct
EIVLTQSPGTLSLSPGERATLSCRASQSVGDFYLAWYQQKPGQAPRLLIYGASSRATGIPDRFSGSGSGTDFTLTISRLEPEDFAVYYCKHYGWPPSFTFGQGTKVEIK

SEQ ID NO: 12 - protein, 109 aa, synthetic construct
  REGION 1..109: note = Synthetic Construct
EIVLTQSPGTLSLSPGERATLSCRASQSVGDFYLAWYQQKPGQAPRLLIYGASSRATGIPDRFSGSGSGTDFTLTISRLEPEDFAVYYCQHYPYPPSFTFGQGTKVEIK

SEQ ID NO: 13 - protein, 109 aa, synthetic construct; identical to SEQ ID NO: 6
  REGION 1..109: note = Synthetic Construct

SEQ ID NO: 14 - protein, 109 aa, synthetic construct; identical to SEQ ID NO: 6
  REGION 1..109: note = Synthetic Construct

SEQ ID NO: 15 - protein, 109 aa, synthetic construct
  REGION 1..109: note = Synthetic Construct
EIVLTQSPGTLSLSPGERATLSCRASQSVSSSYLAWYQQKPGQAPRLLIYGASSRATGIPDRFSGSGSGTDFTLTISRLEPEDFAVYYCKHYGWPPSFTFGQGTKVEIK

SEQ ID NO: 16 - protein, 109 aa, synthetic construct
  REGION 1..109: note = Synthetic Construct
EIVLTQSPGTLSLSPGERATLSCRASQSVSSSYLAWYQQKPGQAPRLLIYGASSRATGIPDRFSGSGSGTDFTLTISRLEPEDFAVYYCQHYPYPPSFTFGQGTKVEIK

SEQ ID NO: 17 - protein, 109 aa, synthetic construct
  REGION 1..109: note = Synthetic Construct
EIVLTQSPGTLSLSPGERATLSCRASQSVSSSYLAWYQQKPGQAPRLLIYGASSRATGIPDRFSGSGSGTDFTLTISRLEPEDFAVYYCQHYNYPPSFTFGQGTKVEIK

SEQ ID NO: 18 - protein, 109 aa, synthetic construct
  REGION 1..109: note = Synthetic Construct
EIVLTQSPGTLSLSPGERATLSCRASQSVSSSYPSWYQQKPGQAPRLLIYGASSRATGIPDRFSGSGSGTDFTLTISRLEPEDFAVYYCQHYPYPPSFTFGQGTKVEIK

SEQ ID NO: 19 - protein, 109 aa, synthetic construct
  REGION 1..109: note = Synthetic Construct
EIVLTQSPGTLSLSPGERATLSCRASQSVSAHYLAWYQQKPGQAPRLLIYGASSRATGIPDRFSGSGSGTDFTLTISRLEPEDFAVYYCQHYPYPPSFTFGQGTKVEIK

SEQ ID NO: 20 - protein, 109 aa, synthetic construct
  REGION 1..109: note = Synthetic Construct
EIVLTQSPGTLSLSPGERATLSCRASQSVSSFFLAWYQQKPGQAPRLLIYGASSRATGIPDRFSGSGSGTDFTLTISRLEPEDFAVYYCQHYPYPPSFTFGQGTKVEIK

SEQ ID NO: 21 - protein, 109 aa, synthetic construct
  REGION 1..109: note = Synthetic Construct
EIVLTQSPGTLSLSPGERATLSCRASQSVSPHYLAWYQQKPGQAPRLLIYGASSRATGIPDRFSGSGSGTDFTLTISRLEPEDFAVYYCQHYPYPPSFTFGQGTKVEIK

SEQ ID NO: 22 - protein, 109 aa, synthetic construct
  REGION 1..109: note = Synthetic Construct
EIVLTQSPGTLSLSPGERATLSCRASQSVSSSYLAWYQQKPGQAPRLLIYGASSRATGIPDRFSGSGSGTDFTLTISRLEPEDFAVYYCKYYPYPPSFTFGQGTKVEIK

SEQ ID NO: 23 - protein, 109 aa, synthetic construct
  REGION 1..109: note = Synthetic Construct
EIVLTQSPGTLSLSPGERATLSCRASQSVSSSYLAWYQQKPGQAPRLLIYGASSRATGIPDRFSGSGSGTDFTLTISRLEPEDFAVYYCKFYPYPPSFTFGQGTKVEIK

SEQ ID NO: 24 - protein, 119 aa, synthetic construct
  REGION 1..119: note = Synthetic Construct
EVQLLESGGGLVQPGGSLRLSCAASGFTFGSYAMTWVRQAPGKGLEWVSAISGSGGNTFYADQRKGRFTISRDNSKNTLYLQMNSLRAEDTAVYYCARVSPIASGMDYWGQGTLVTVSS

SEQ ID NO: 25 - protein, 119 aa, synthetic construct
  REGION 1..119: note = Synthetic Construct
EVQLLESGGGLVQPGGSLRLSCAASGFTFGSYAMTWVRQAPGKGLEWVSAIDYSGGNTFYADSVKGRFTISRDNSKNTLYLQMNSLRAEDTAVYYCARVSPIASGMDYWGQGTLVTVSS

SEQ ID NO: 26 - protein, 119 aa, synthetic construct
  REGION 1..119: note = Synthetic Construct
EVQLLESGGGLVQPGGSLRLSCAASGFTFGSYAMTWVRQAPGKGLEWVSAISYQGGNTFYADSVKGRFTISRDNSKNTLYLQMNSLRAEDTAVYYCARVSPIASGMDYWGQGTLVTVSS

SEQ ID NO: 27 - protein, 119 aa, synthetic construct
  REGION 1..119: note = Synthetic Construct
EVQLLESGGGLVQPGGSLRLSCAASGFTFGSYAMTWVRQAPGKGLEWVSAISLTGGNTFYADSVKGRFTISRDNSKNTLYLQMNSLRAEDTAVYYCARVSPIASGMDYWGQGTLVTVSS

SEQ ID NO: 28 - protein, 119 aa, synthetic construct
  REGION 1..119: note = Synthetic Construct
EVQLLESGGGLVQPGGSLRLSCAASGFTFGSYAMTWVRQAPGKGLEWVSAISHAGGNTFYADSVKGRFTISRDNSKNTLYLQMNSLRAEDTAVYYCARVSPIASGMDYWGQGTLVTVSS

SEQ ID NO: 29 - protein, 119 aa, synthetic construct
  REGION 1..119: note = Synthetic Construct
EVQLLESGGGLVQPGGSLRLSCAASGFTFGSYAMTWVRQAPGKGLEWVSAISGSGGNTFYADQLKGRFTISRDNSKNTLYLQMNSLRAEDTAVYYCARVSPIASGMDYWGQGTLVTVSS

SEQ ID NO: 30 - protein, 119 aa, synthetic construct
  REGION 1..119: note = Synthetic Construct
EVQLLESGGGLVQPGGSLRLSCAASGFTFGSYAMTWVRQAPGKGLEWVSAISGSGGNTFYADSVKGRFTISRDNSKNTLYLQMNSLRAEDTAVYYCARVSPIYAGMDYWGQGTLVTVSS

SEQ ID NO: 31 - protein, 119 aa, synthetic construct
  REGION 1..119: note = Synthetic Construct
EVQLLESGGGLVQPGGSLRLSCAASGFTFGSYAMTWVRQAPGKGLEWVSAISGSGGNTFYADSVKGRFTISRDNSKNTLYLQMNSLRAEDTAVYYCARVSPIAAEMDYWGQGTLVTVSS

SEQ ID NO: 32 - protein, 119 aa, synthetic construct
  REGION 1..119: note = Synthetic Construct
EVQLLESGGGLVQPGGSLRLSCAASGFTFGSYAMTWVRQAPGKGLEWVSAISGSGGNTFYADSVKGRFTISRDNSKNTLYLQMNSLRAEDTAVYYCTRVSPIAAQMDYWGQGTLVTVSS

SEQ ID NO: 33 - protein, 115 aa, synthetic construct
  REGION 1..115: note = Synthetic Construct
EVQLLESGGGLVQPGGSLRLSCAASGFTFSSYAMNWVRQAPGKGLEWVSAISDSGGSTYYADSVKGRFTISRDNSKNTLYLQMNSLRAEDTAVYYCARYWPMDIWGQGTLVTVSS

SEQ ID NO: 34 - protein, 108 aa, synthetic construct
  REGION 1..108: note = Synthetic Construct
EIVLTQSPGTLSLSPGERATLSCRASQSVSSSYLAWYQQKPGQAPRLLMYDASIRATGIPDRFSGSGSGTDFTLTISRLEPEDFAVYYCQQYGSWPLTFGQGTKVEIK

SEQ ID NO: 35 - protein, 115 aa, synthetic construct
  REGION 1..115: note = Synthetic Construct
EVQLLESGGGLVQPGGSLRLSCAASGFTFSSYAMNWVRQAPGKGLEWVSAISDSGGSAWYADSVKGRFTISRDNSKNTLYLQMNSLRAEDTAVYYCARYWPMSLWGQGTLVTVSS

SEQ ID NO: 36 - protein, 108 aa, synthetic construct
  REGION 1..108: note = Synthetic Construct
EIVLTQSPGTLSLSPGERATLSCRASQSVSVLYLAWYQQKPGQAPRLLMYDASIRATGIPDRFSGSGSGTDFTLTISRLEPEDFAVYYCQQYQRWPLTFGQGTKVEIK

SEQ ID NO: 37 - protein, 115 aa, synthetic construct
  REGION 1..115: note = Synthetic Construct
EVQLLESGGGLVQPGGSLRLSCAASGFTFSSYAMNWVRQAPGKGLEWVSAISDSGGSMWYADSVKGRFTISRDNSKNTLYLQMNSLRAEDTAVYYCARYWPMSLWGQGTLVTVSS

SEQ ID NO: 38 - protein, 108 aa, synthetic construct
  REGION 1..108: note = Synthetic Construct
EIVLTQSPGTLSLSPGERATLSCRASQSVSSSYLAWYQQKPGQAPRLLMYDASIRATGIPDRFSGSGSGTDFTLTISRLEPEDFAVYYCQQYQSWPLTFGQGTKVEIK

SEQ ID NO: 39 - protein, 115 aa, synthetic construct
  REGION 1..115: note = Synthetic Construct
EVQLLESGGGLVQPGGSLRLSCAASGFTFSSYAMNWVRQAPGKGLEWVSAISDFGGSTYYADSVKGRFTISRDNSKNTLYLQMNSLRAEDTAVYYCARYWPMDIWGQGTLVTVSS

SEQ ID NO: 40 - protein, 108 aa, synthetic construct
  REGION 1..108: note = Synthetic Construct
EIVLTQSPGTLSLSPGERATLSCRASQSVSDLYLAWYQQKPGQAPRLLMYDASIRATGIPDRFSGSGSGTDFTLTISRLEPEDFAVYYCQQYQTWPLTFGQGTKVEIK

SEQ ID NO: 41 - protein, 108 aa, synthetic construct
  REGION 1..108: note = Synthetic Construct
EIVLTQSPGTLSLSPGERATLSCRASQSVSNLYLAWYQQKPGQAPRLLMYDASIRATGIPDRFSGSGSGTDFTLTISRLEPEDFAVYYCQQYQGWPLTFGQGTKVEIK

SEQ ID NO: 42 - protein, 115 aa, synthetic construct
  REGION 1..115: note = Synthetic Construct
EVQLLESGGGLVQPGGSLRLSCAASGFTFSSYAMNWVRQAPGKGLEWVSAITASGGSTYYADSVKGRFTISRDNSKNTLYLQMNSLRAEDTAVYYCARYWPMSLWGQGTLVTVSS

SEQ ID NO: 43 - protein, 108 aa, synthetic construct
  REGION 1..108: note = Synthetic Construct
EIVLTQSPGTLSLSPGERATLSCRASQSVSAYYLAWYQQKPGQAPRLLMYDASIRATGIPDRFSGSGSGTDFTLTISRLEPEDFAVYYCQQYERWPLTFGQGTKVEIK

SEQ ID NO: 44 - protein, 115 aa, synthetic construct
  REGION 1..115: note = Synthetic Construct
EVQLLESGGGLVQPGGSLRLSCAASGFTFSSYAMNWVRQAPGKGLEWVSAISDSGGSTYYADSVKGRFTISRDNSKNTLYLQMNSLRAEDTAVYYCARYWPMSLWGQGTLVTVSS

SEQ ID NO: 45 - protein, 108 aa, synthetic construct
  REGION 1..108: note = Synthetic Construct
EIVLTQSPGTLSLSPGERATLSCRASQSVSSLYLAWYQQKPGQAPRLLMYDASIRATGIPDRFSGSGSGTDFTLTISRLEPEDFAVYYCQQYQVWPLTFGQGTKVEIK

SEQ ID NO: 46 - protein, 115 aa, synthetic construct
  REGION 1..115: note = Synthetic Construct
EVQLLESGGGLVQPGGSLRLSCAASGFTFSSYAMNWVRQAPGKGLEWVSAISDSGGSRWYADSVKGRFTISRDNSKNTLYLQMNSLRAEDTAVYYCARYWPMTPWGQGTLVTVSS

SEQ ID NO: 47 - protein, 108 aa, synthetic construct
  REGION 1..108: note = Synthetic Construct
EIVLTQSPGTLSLSPGERATLSCRASQSVSSSYLAWYQQKPGQAPRLLMYDASIRATGIPDRFSGSGSGTDFTLTISRLEPEDFAVYYCQQYLDWPLTFGQGTKVEIK

SEQ ID NO: 48 - protein, 115 aa, synthetic construct
  REGION 1..115: note = Synthetic Construct
EVQLLESGGGLVQPGGSLRLSCAASGFTFSSYAMNWVRQAPGKGLEWVSAVLDSGGSTYYADSVKGRFTISRDNSKNTLYLQMNSLRAEDTAVYYCARYWPMTPWGQGTLVTVSS

SEQ ID NO: 49 - protein, 108 aa, synthetic construct
  REGION 1..108: note = Synthetic Construct
EIVLTQSPGTLSLSPGERATLSCRASQSVSSSYLAWYQQKPGQAPRLLMYDASIRATGIPDRFSGSGSGTDFTLTISRLEPEDFAVYYCQQYQVWPLTFGQGTKVEIK

SEQ ID NO: 50 - protein, 115 aa, synthetic construct
  REGION 1..115: note = Synthetic Construct
EVQLLESGGGLVQPGGSLRLSCAASGFTFSSYAMNWVRQAPGKGLEWVSAISDSGGSRWYADSVKGRFTISRDNSKNTLYLQMNSLRAEDTAVYYCARYWPMSDWGQGTLVTVSS

SEQ ID NO: 51 - protein, 108 aa, synthetic construct
  REGION 1..108: note = Synthetic Construct
EIVLTQSPGTLSLSPGERATLSCRASQSVSVLYLAWYQQKPGQAPRLLMYDASIRATGIPDRFSGSGSGTDFTLTISRLEPEDFAVYYCQQYLAWPLTFGQGTKVEIK

SEQ ID NO: 52 - protein, 115 aa, synthetic construct
  REGION 1..115: note = Synthetic Construct
EVQLLESGGGLVQPGGSLRLSCAASGFTFSSYAMNWVRQAPGKGLEWVSAISDSGGSKWYADSVKGRFTISRDNSKNTLYLQMNSLRAEDTAVYYCARYWPMSLWGQGTLVTVSS

SEQ ID NO: 53 - protein, 108 aa, synthetic construct
  REGION 1..108: note = Synthetic Construct
EIVLTQSPGTLSLSPGERATLSCRASQSVSSSYLAWYQQKPGQAPRLLMYDASIRATGIPDRFSGSGSGTDFTLTISRLEPEDFAVYYCQQYFTWPLTFGQGTKVEIK

SEQ ID NO: 54 - protein, 115 aa, synthetic construct
  REGION 1..115: note = Synthetic Construct
EVQLLESGGGLVQPGGSLRLSCAASGFTFSSYAMNWVRQAPGKGLEWVSAIGGSGGSLPYADSVKGRFTISRDNSKNTLYLQMNSLRAEDTAVYYCARYWPMDSWGQGTLVTVSS

SEQ ID NO: 55 - protein, 108 aa, synthetic construct
  REGION 1..108: note = Synthetic Construct
EIVLTQSPGTLSLSPGERATLSCRASQSVSPYYLAWYQQKPGQAPRLLMYDASIRATGIPDRFSGSGSGTDFTLTISRLEPEDFAVYYCQQYERWPLTFGQGTKVEIK

SEQ ID NO: 56 - protein, 115 aa, synthetic construct
  REGION 1..115: note = Synthetic Construct
EVQLLESGGGLVQPGGSLRLSCAASGFTFSSYAMNWVRQAPGKGLEWVSAISDSGGSGWYADSVKGRFTISRDNSKNTLYLQMNSLRAEDTAVYYCARYWPMSLWGQGTLVTVSS

SEQ ID NO: 57 - protein, 108 aa, synthetic construct
  REGION 1..108: note = Synthetic Construct
EIVLTQSPGTLSLSPGERATLSCRASQSVSVEYLAWYQQKPGQAPRLLMYDASIRATGIPDRFSGSGSGTDFTLTISRLEPEDFAVYYCQQYARWPLTFGQGTKVEIK

SEQ ID NO: 58 - protein, 115 aa, synthetic construct
  REGION 1..115: note = Synthetic Construct
EVQLLESGGGLVQPGGSLRLSCAASGFTFSSYAMNWVRQAPGKGLEWVSAVLDSGGSTYYADSVKGRFTISRDNSKNTLYLQMNSLRAEDTAVYYCARYWPMSLWGQGTLVTVSS

SEQ ID NO: 59 - protein, 108 aa, synthetic construct
  REGION 1..108: note = Synthetic Construct
EIVLTQSPGTLSLSPGERATLSCRASQSVSELYLAWYQQKPGQAPRLLMYDASIRATGIPDRFSGSGSGTDFTLTISRLEPEDFAVYYCQQYFGWPLTFGQGTKVEIK

SEQ ID NO: 60 - protein, 115 aa, synthetic construct
  REGION 1..115: note = Synthetic Construct
EVQLLESGGGLVQPGGSLRLSCAASGFTFSSYAMNWVRQAPGKGLEWVSAISDSGGSCWYADSVKGRFTISRDNSKNTLYLQMNSLRAEDTAVYYCARYWPMTPWGQGTLVTVSS

SEQ ID NO: 61 - protein, 108 aa, synthetic construct
  REGION 1..108: note = Synthetic Construct
EIVLTQSPGTLSLSPGERATLSCRASQSVEMSYLAWYQQKPGQAPRLLMYDASIRATGIPDRFSGSGSGTDFTLTISRLEPEDFAVYYCQQYAHWPLTFGQGTKVEIK

SEQ ID NO: 62 - protein, 115 aa, synthetic construct
  REGION 1..115: note = Synthetic Construct
EVQLLESGGGLVQPGGSLRLSCAASGFTFSSYAMNWVRQAPGKGLEWVSAIFASGGSTYYADSVKGRFTISRDNSKNTLYLQMNSLRAEDTAVYYCARYWPMTPWGQGTLVTVSS

SEQ ID NO: 63 - protein, 108 aa, synthetic construct
  REGION 1..108: note = Synthetic Construct
EIVLTQSPGTLSLSPGERATLSCRASQSVSSSYLAWYQQKPGQAPRLLMYDASIRATGIPDRFSGSGSGTDFTLTISRLEPEDFAVYYCQQYQRWPLTFGQGTKVEIK

SEQ ID NO: 64 - protein, 115 aa, synthetic construct
  REGION 1..115: note = Synthetic Construct
EVQLLESGGGLVQPGGSLRLSCAASGFTFSSYAMNWVRQAPGKGLEWVSAISGWGGSLPYADSVKGRFTISRDNSKNTLYLQMNSLRAEDTAVYYCARYWPMDSWGQGTLVTVSS

SEQ ID NO: 65 - protein, 108 aa, synthetic construct
  REGION 1..108: note = Synthetic Construct
EIVLTQSPGTLSLSPGERATLSCRASQSVSAQYLAWYQQKPGQAPRLLMYDASIRATGIPDRFSGSGSGTDFTLTISRLEPEDFAVYYCQQYQRWPLTFGQGTKVEIK

SEQ ID NO: 66 - protein, 115 aa, synthetic construct
  REGION 1..115: note = Synthetic Construct
EVQLLESGGGLVQPGGSLRLSCAASGFTFSSYAMNWVRQAPGKGLEWVSAIMSSGGPLYYADSVKGRFTISRDNSKNTLYLQMNSLRAEDTAVYYCARYWPMALWGQGTLVTVSS

SEQ ID NO: 67 - protein, 108 aa, synthetic construct
  REGION 1..108: note = Synthetic Construct
EIVLTQSPGTLSLSPGERATLSCRASQSVSALYLAWYQQKPGQAPRLLMYDASIRATGIPDRFSGSGSGTDFTLTISRLEPEDFAVYYCQQYQVWPLTFGQGTKVEIK

SEQ ID NO: 68 - protein, 115 aa, synthetic construct
  REGION 1..115: note = Synthetic Construct
EVQLLESGGGLVQPGGSLRLSCAASGFTFSSYAMNWVRQAPGKGLEWVSAILMSGGSTYYADSVKGRFTISRDNSKNTLYLQMNSLRAEDTAVYYCARYWPMSLWGQGTLVTVSS

SEQ ID NO: 69 - protein, 108 aa, synthetic construct
  REGION 1..108: note = Synthetic Construct
EIVLTQSPGTLSLSPGERATLSCGPSQSVSSSYLAWYQQKPGQAPRLLMYDASIRATGIPDRFSGSGSGTDFTLTISRLEPEDFAVYYCQQYQSWPLTFGQGTKVEIK

SEQ ID NO: 70 - protein, 115 aa, synthetic construct
  REGION 1..115: note = Synthetic Construct
EVQLLESGGGLVQPGGSLRLSCAASGFTFSSYAMNWVRQAPGKGLEWVSAISDSGGYRYYADSVKGRFTISRDNSKNTLYLQMNSLRAEDTAVYYCARYWPMSLWGQGTLVTVSS

SEQ ID NO: 71 - protein, 108 aa, synthetic construct
  REGION 1..108: note = Synthetic Construct
EIVLTQSPGTLSLSPGERATLSCRASQSVSSSYWAWYQQKPGQAPRLLMYDASIRATGIPDRFSGSGSGTDFTLTISRLEPEDFAVYYCQQYESWPLTFGQGTKVEIK

SEQ ID NO: 72 - protein, 115 aa, synthetic construct
  REGION 1..115: note = Synthetic Construct
EVQLLESGGGLVQPGGSLRLSCAASGFTFSSYAMNWVRQAPGKGLEWVSAILSSGGSTYYADSVKGRFTISRDNSKNTLYLQMNSLRAEDTAVYYCARYWPMDIWGQGTLVTVSS

SEQ ID NO: 73 - protein, 108 aa, synthetic construct
  REGION 1..108: note = Synthetic Construct
EIVLTQSPGTLSLSPGERATLSCRGGQSVSSSYLAWYQQKPGQAPRLLMYDASIRATGIPDRFSGSGSGTDFTLTISRLEPEDFAVYYCQQYQSWPLTFGQGTKVEIK

SEQ ID NO: 74 - protein, 115 aa, synthetic construct
  REGION 1..115: note = Synthetic Construct
EVQLLESGGGLVQPGGSLRLSCAASGFTFSSYAMNWVRQAPGKGLEWVSAILDSGGSTYYADSVKGRFTISRDNSKNTLYLQMNSLRAEDTAVYYCARYWPMSPWGQGTLVTVSS

SEQ ID NO: 75 - protein, 108 aa, synthetic construct
  REGION 1..108: note = Synthetic Construct
EIVLTQSPGTLSLSPGERATLSCRASQSVSFLYLAWYQQKPGQAPRLLMYDASIRATGIPDRFSGSGSGTDFTLTISRLEPEDFAVYYCQQYGSWPLTFGQGTKVEIK

SEQ ID NO: 76 - protein, 115 aa, synthetic construct
  REGION 1..115: note = Synthetic Construct
EVQLLESGGGLVQPGGSLRLSCAASGFTFSSYPMSWVRQAPGKGLEWVSAIGGSGGSTYYADSVKGRFTISRDNSKNTLYLQMNSLRAEDTAVYYCARYWPMDSWGQGTLVTVSS

SEQ ID NO: 77 - protein, 108 aa, synthetic construct
  REGION 1..108: note = Synthetic Construct
EIVLTQSPGTLSLSPGERATLSCRASQSVSSTYLAWYQQKPGQAPRLLIYDASSRAPGIPDRFSGSGSGTDFTLTISRLEPEDFAVYYCQQYSTSPLTFGQGTKVEIK

SEQ ID NO: 78 - protein, 115 aa, synthetic construct
  REGION 1..115: note = Synthetic Construct
EVQLLESGGGLVQPGGSLRLSCAASGFTFSSYPMSWVRQAPGKGLEWVSAIGGSGGSLPYADSVKGRFTISRDNSKNTLYLQMNSLRAEDTAVYYCARYWPMDSWGQGTLVTVSS

SEQ ID NO: 79 - protein, 108 aa, synthetic construct
  REGION 1..108: note = Synthetic Construct
EIVLTQSPGTLSLSPGERATLSCRASQSVSPEYLAWYQQKPGQAPRLLIYDASSRAPGIPDRFSGSGSGTDFTLTISRLEPEDFAVYYCQQYSVWPLTFGQGTKVEIK

SEQ ID NO: 80 - protein, 109 aa, synthetic construct
  REGION 1..109: note = Synthetic Construct
EIVLTQSPGTLSLSPGERATLSCRASQSVSSSYLAWYQQKPGQAPRLLIYGASSRAYGIPDRFSGSGSGTDFTLTISRLEPEDFAVYYCQHYGSPPLFTFGQGTKVEIK

SEQ ID NO: 81 - protein, 108 aa, synthetic construct
  REGION 1..108: note = Synthetic Construct
EIVLTQSPGTLSLSPGERATLSCRASQSVSSTYLAWYQQKPGQAPRLLIYDASSRAPGIPDRFSGSGSGTDFTLTISRLEPEDFAVYYCQQYSRWPLTFGQGTKVEIK

SEQ ID NO: 82 - protein, 108 aa, synthetic construct
  REGION 1..108: note = Synthetic Construct
EIVLTQSPGTLSLSPGERATLSCRASQSVSPLYLAWYQQKPGQAPRLLIYDASSRAPGIPDRFSGSGSGTDFTLTISRLEPEDFAVYYCQQYSAFPLTFGQGTKVEIK

SEQ ID NO: 83 - protein, 115 aa, synthetic construct
  REGION 1..115: note = Synthetic Construct
EVQLLESGGGLVQPGGSLRLSCAASGFTFSSYPMSWVRQAPGKGLEWVSAIGGSGGWSYYADSVKGRFTISRDNSKNTLYLQMNSLRAEDTAVYYCARYWPMDSWGQGTLVTVSS

SEQ ID NO: 84 - protein, 108 aa, synthetic construct
  REGION 1..108: note = Synthetic Construct
EIVLTQSPGTLSLSPGERATLSCWLSQSVSSTYLAWYQQKPGQAPRLLIYDASSRAPGIPDRFSGSGSGTDFTLTISRLEPEDFAVYYCQQYSEWPLTFGQGTKVEIK

SEQ ID NO: 85 - protein, 108 aa, synthetic construct
  REGION 1..108: note = Synthetic Construct
EIVLTQSPGTLSLSPGERATLSCRASQSVSSTYLAWYQQKPGQAPRLLIYDASSRAPGIPDRFSGSGSGTDFTLTISRLEPEDFAVYYCQQYSSWPLTFGQGTKVEIK

SEQ ID NO: 86 - protein, 108 aa, synthetic construct
  REGION 1..108: note = Synthetic Construct
EIVLTQSPGTLSLSPGERATLSCRASQSVSSLFLAWYQQKPGQAPRLLIYDASSRAPGIPDRFSGSGSGTDFTLTISRLEPEDFAVYYCQQYSAWPLTFGQGTKVEIK

SEQ ID NO: 87 - protein, 115 aa, synthetic construct
  REGION 1..115: note = Synthetic Construct
EVQLLESGGGLVQPGGSLRLSCAASGFTFSSYPMSWVRQAPGKGLEWVSATVGSGGSIGYADSVKGRFTISRDNSKNTLYLQMNSLRAEDTAVYYCARYWPMDSWGQGTLVTVSS

SEQ ID NO: 88 - protein, 108 aa, synthetic construct
  REGION 1..108: note = Synthetic Construct
EIVLTQSPGTLSLSPGERATLSCACSQSVSSTYLAWYQQKPGQAPRLLIYDASSRAPGIPDRFSGSGSGTDFTLTISRLEPEDFAVYYCQQYSAWPLTFGQGTKVEIK

SEQ ID NO: 89 - protein, 108 aa, synthetic construct
  REGION 1..108: note = Synthetic Construct
EIVLTQSPGTLSLSPGERATLSCRASCDVSSTYLAWYQQKPGQAPRLLIYDASSRAPGIPDRFSGSGSGTDFTLTISRLEPEDFAVYYCQQYMRSPLTFGQGTKVEIK

SEQ ID NO: 90 - protein, 108 aa, synthetic construct
  REGION 1..108: note = Synthetic Construct
EIVLTQSPGTLSLSPGERATLSCRASEAVPSTYLAWYQQKPGQAPRLLIYDASSRAPGIPDRFSGSGSGTDFTLTISRLEPEDFAVYYCQQYSAFPLTFGQGTKVEIK

SEQ ID NO: 91 - protein, 108 aa, synthetic construct
  REGION 1..108: note = Synthetic Construct
EIVLTQSPGTLSLSPGERATLSCCSSQSVSSTYLAWYQQKPGQAPRLLIYDASSRAPGIPDRFSGSGSGTDFTLTISRLEPEDFAVYYCQQYSAFPLTFGQGTKVEIK

SEQ ID NO: 92 - protein, 115 aa, synthetic construct
  REGION 1..115: note = Synthetic Construct
EVQLLESGGGLVQPGGSLRLSCAASGFTFSSYAMNWVRQAPGKGLEWVSAISDSGGSRWYADSVKGRFTISRDNSKNTLYLQMNSLRAEDTAVYYCTRYWPMDIWGQGTLVTVSS

SEQ ID NO: 93 - protein, 108 aa, synthetic construct
  REGION 1..108: note = Synthetic Construct
EIVLTQSPGTLSLSPGERATLSCRASVRVSSTYLAWYQQKPGQAPRLLMYDASIRATGIPDRFSGSGSGTDFTLTISRLEPEDFAVYYCQQYMKWPLTFGQGTKVEIK

SEQ ID NO: 94 - protein, 108 aa, synthetic construct
  REGION 1..108: note = Synthetic Construct
EIVLTQSPGTLSLSPGERATLSCRASQSVSAAYLAWYQQKPGQAPRLLMYDASIRATGIPDRFSGSGSGTDFTLTISRLEPEDFAVYYCQQYMCWPLTFGQGTKVEIK

SEQ ID NO: 95 - protein, 115 aa, synthetic construct
  REGION 1..115: note = Synthetic Construct
EVQLLESGGGLVQPGGSLRLSCAASGFTFSSYPMSWVRQAPGKGLEWVSAIGGSGGSIHYADSVKGRFTISRDNSKNTLYLQMNSLRAEDTAVYYCARYWPMDSWGQGTLVTVSS

SEQ ID NO: 96 - protein, 108 aa, synthetic construct
  REGION 1..108: note = Synthetic Construct
EIVLTQSPGTLSLSPGERATLSCRASQSVSSSYWGWYQQKPGQAPRLLMYDASIRATGIPDRFSGSGSGTDFTLTISRLEPEDFAVYYCQQYQCWPLTFGQGTKVEIK

SEQ ID NO: 97 - protein, 115 aa, synthetic construct
  REGION 1..115: note = Synthetic Construct
EVQLLESGGGLVQPGGSLRLSCAASGFTFSSYPMSWVRQAPGKGLEWVSAHIGSGGSTYYADSVKGRFTISRDNSKNTLYLQMNSLRAEDTAVYYCARYWPMDSWGQGTLVTVSS

SEQ ID NO: 98 - protein, 108 aa, synthetic construct
  REGION 1..108: note = Synthetic Construct
EIVLTQSPGTLSLSPGERATLSCRASQSVSSTYLAWYQQKPGQAPRLLMYDASIRATGIPDRFSGSGSGTDFTLTISRLEPEDFAVYYCQQYQSWPLTFGQGTKVEIK

SEQ ID NO: 99 - protein, 115 aa, synthetic construct
  REGION 1..115: note = Synthetic Construct
EVQLLESGGGLVQPGGSLRLSCAASGFTFSSYPMSWVRQAPGKGLEWVSAIGGSGGSTYYADSVKGRFTISRDNSKNTLYLQMNSLRAEDTAVYYCARYWPMDPWGQGTLVTVSS

SEQ ID NO: 100 - protein, 108 aa, synthetic construct
  REGION 1..108: note = Synthetic Construct
EIVLTQSPGTLSLSPGERATLSCRASQSVSSPYLAWYQQKPGQAPRLLMYDASIRATGIPDRFSGSGSGTDFTLTISRLEPEDFAVYYCQQYQSWPLTFGQGTKVEIK

SEQ ID NO: 101 - protein, 115 aa, synthetic construct
  REGION 1..115: note = Synthetic Construct
EVQLLESGGGLVQPGGSLRLSCAASGFTFSSYPMSWVRQAPGKGLEWVSAIGGSGGSLGYADSVKGRFTISRDNSKNTLYLQMNSLRAEDTAVYYCARYWPMDSWGQGTLVTVSS

SEQ ID NO: 102 - protein, 108 aa, synthetic construct
  REGION 1..108: note = Synthetic Construct
EIVLTQSPGTLSLSPGERATLSCRASQSVSPLYLAWYQQKPGQAPRLLMYDASIRATGIPDRFSGSGSGTDFTLTISRLEPEDFAVYYCQQYKAWPLTFGQGTKVEIK

SEQ ID NO: 103 - protein, 108 aa, synthetic construct
  REGION 1..108: note = Synthetic Construct
EIVLTQSPGTLSLSPGERATLSCRASQSVSYLYLAWYQQKPGQAPRLLMYDASIRATGIPDRFSGSGSGTDFTLTISRLEPEDFAVYYCQQYMEWPLTFGQGTKVEIK

SEQ ID NO: 104 - protein, 115 aa, synthetic construct
  REGION 1..115: note = Synthetic Construct
EVQLLESGGGLVQPGGSLRLSCAASGFTFSSYPMSWVRQAPGKGLEWVSAIFASGGSTYYADSVKGRFTISRDNSKNTLYLQMNSLRAEDTAVYYCARYWPMDSWGQGTLVTVSS

SEQ ID NO: 105 - protein, 108 aa, synthetic construct
  REGION 1..108: note = Synthetic Construct
EIVLTQSPGTLSLSPGERATLSCRASQSVSAQYLAWYQQKPGQAPRLLMYDASIRATGIPDRFSGSGSGTDFTLTISRLEPEDFAVYYCQQYQAWPLTFGQGTKVEIK

SEQ ID NO: 106 - protein, 115 aa, synthetic construct
  REGION 1..115: note = Synthetic Construct
EVQLLESGGGLVQPGGSLRLSCAASGFTFSSYPMSWVRQAPGKGLEWVSAIGGSGTWTYYADSVKGRFTISRDNSKNTLYLQMNSLRAEDTAVYYCARYWPMDSWGQGTLVTVSS

SEQ ID NO: 107 - protein, 108 aa, synthetic construct
  REGION 1..108: note = Synthetic Construct
EIVLTQSPGTLSLSPGERATLSCRASQSVSSSYLAWYQQKPGQAPRLLMYDASIRATGIPDRFSGSGSGTDFTLTISRLEPEDFAVYYCQQYQKWPLTFGQGTKVEIK

SEQ ID NO: 108 - protein, 108 aa, synthetic construct
  REGION 1..108: note = Synthetic Construct
EIVLTQSPGTLSLSPGERATLSCRASQSVSAVYLAWYQQKPGQAPRLLMYDASIRATGIPDRFSGSGSGTDFTLTISRLEPEDFAVYYCQQYRAWPLTFGQGTKVEIK

SEQ ID NO: 109 - protein, 108 aa, synthetic construct
  REGION 1..108: note = Synthetic Construct
EIVLTQSPGTLSLSPGERATLSCRASIAVSSTYLAWYQQKPGQAPRLLMYDASIRATGIPDRFSGSGSGTDFTLTISRLEPEDFAVYYCQQYMVWPLTFGQGTKVEIK

SEQ ID NO: 110 - protein, 115 aa, synthetic construct
  REGION 1..115: note = Synthetic Construct
EVQLLESGGGLVQPGGSLRLSCAASGFTFSSYPMSWVRQAPGKGLEWVSALFGSGGSTYYADSVKGRFTISRDNSKNTLYLQMNSLRAEDTAVYYCARYWPMDSWGQGTLVTVSS

SEQ ID NO: 111 - protein, 108 aa, synthetic construct
  REGION 1..108: note = Synthetic Construct
EIVLTQSPGTLSLSPGERATLSCRPRQSVSSSYLAWYQQKPGQAPRLLMYDASIRATGIPDRFSGSGSGTDFTLTISRLEPEDFAVYYCQQYQDWPLTFGQGTKVEIK

SEQ ID NO: 112 - protein, 115 aa, synthetic construct
  REGION 1..115: note = Synthetic Construct
EVQLLESGGGLVQPGGSLRLSCAASGFTFSSYPMSWVRQAPGKGLEWVSAIGGSGGSLPYADSVKGRFTISRDNSKNTLYLQMNSLRAEDTAVYYCARYWPMDIWGQGTLVTVSS

SEQ ID NO: 113 - protein, 108 aa, synthetic construct
  REGION 1..108: note = Synthetic Construct
EIVLTQSPGTLSLSPGERATLSCRASQSVSSTYLAWYQQKPGQAPRLLMYDASIRATGIPDRFSGSGSGTDFTLTISRLEPEDFAVYYCQQYQEWPLTFGQGTKVEIK

SEQ ID NO: 114 - protein, 114 aa, synthetic construct
  REGION 1..114: note = Synthetic Construct
EVQLLESGGGLVQPGGSLRLSCAASGFTFSSYPMSWVRQAPGKGLEWVSAALGSGGSTYYADSVKGRFTISRDNSKNTLYLQMNSLRAEDTAVYYCARYWPMDSWGQGTLVTVS

SEQ ID NO: 115 - protein, 108 aa, synthetic construct
  REGION 1..108: note = Synthetic Construct
EIVLTQSPGTLSLSPGERATLSCRASQSVSASYLAWYQQKPGQAPRLLMYDASIRATGIPDRFSGSGSGTDFTLTISRLEPEDFAVYYCQQYMSWPLTFGQGTKVEIK

SEQ ID NO: 116 - protein, 108 aa, synthetic construct
  REGION 1..108: note = Synthetic Construct
EIVLTQSPGTLSLSPGERATLSCRASQSVSYMYLAWYQQKPGQAPRLLIYDASIRATGIPDRFSGSGSGTDFTLTISRLEPEDFAVYYCQQYKSWPLTFGQGTKVEIK

SEQ ID NO: 117 - protein, 108 aa, synthetic construct
  REGION 1..108: note = Synthetic Construct
EIVLTQSPGTLSLSPGERATLSCRASQSVSALYLAWYQQKPGQAPRLLMYDASIRATGIPDRFSGSGSGTDFTLTISRLEPEDFAVYYCQQYYGWPLTFGQGTKVEIK

SEQ ID NO: 118 - protein, 115 aa, synthetic construct
  REGION 1..115: note = Synthetic Construct
EVQLLESGGGLVQPGGSLRLSCAASGFTFSSYPMSWVRQAPGKGLEWVSAIGGSGGSLPYADSVKGRFTISRDNSKNTLYLQMNSLRAEDTAVYYCARYWPMADWGQGTLVTVSS

SEQ ID NO: 119 - protein, 108 aa, synthetic construct
  REGION 1..108: note = Synthetic Construct
EIVLTQSPGTLSLSPGERATLSCRASQPISSSYLAWYQQKPGQAPRLLMYDASIRATGIPDRFSGSGSGTDFTLTISRLEPEDFAVYYCQQYQGWPLTFGQGTKVEIK

SEQ ID NO: 120 - protein, 115 aa, synthetic construct
  REGION 1..115: note = Synthetic Construct
EVQLLESGGGLVQPGGSLRLSCAASGFTFSSYAMNWVRQAPGKGLEWVSAISDSGGFVYYADSVKGRFTISRDNSKNTLYLQMNSLRAEDTAVYYCARYWPMDSWGQGTLVTVSS

SEQ ID NO: 121 - protein, 108 aa, synthetic construct
  REGION 1..108: note = Synthetic Construct
EIVLTQSPGTLSLSPGERATLSCRASQSVSSSYLAWYQQKPGQAPRLLMYDASIRATGIPDRFSGSGSGTDFTLTISRLEPEDFAVYYCQQYEFWPLTFGQGTKVEIK

SEQ ID NO: 122 - protein, 115 aa, synthetic construct
  REGION 1..115: note = Synthetic Construct
EVQLLESGGGLVQPGGSLRLSCAASGFTFSSYAMNWVRQAPGKGLEWVSAIGGSGGSTYYADSVKGRFTISRDNSKNTLYLQMNSLRAEDTAVYYCARYWPMSLWGQGTLVTVSS

SEQ ID NO: 123 - protein, 108 aa, synthetic construct
  REGION 1..108: note = Synthetic Construct
EIVLTQSPGTLSLSPGERATLSCRASQSVSSTYLAWYQQKPGQAPRLLMYDASIRATGIPDRFSGSGSGTDFTLTISRLEPEDFAVYYCQQYMSWPLTFGQGTKVEIK

SEQ ID NO: 124 - protein, 108 aa, synthetic construct
  REGION 1..108: note = Synthetic Construct
EIVLTQSPGTLSLSPGERATLSCRASQGISSTYLAWYQQKPGQAPRLLMYDASIRATGIPDRFSGSGSGTDFTLTISRLEPEDFAVYYCQQYAYWPLTFGQGTKVEIK

SEQ ID NO: 125 - protein, 115 aa, synthetic construct
  REGION 1..115: note = Synthetic Construct
EVQLLESGGGLVQPGGSLRLSCAASGFTFSSYAMNWVRQAPGKGLEWVSACLDSGGSTYYADSVKGRFTISRDNSKNTLYLQMNSLRAEDTAVYYCARYWPMDSWGQGTLVTVSS

SEQ ID NO: 126 - protein, 108 aa, synthetic construct
  REGION 1..108: note = Synthetic Construct
EIVLTQSPGTLSLSPGERATLSCRASQSVSSSYLAWYQQKPGQAPRLLMYDASIRATGIPDRFSGSGSGTDFTLTISRLEPEDFAVYYCQQYQGWPLTFGQGTKVEIK

SEQ ID NO: 127 - protein, 115 aa, synthetic construct
  REGION 1..115: note = Synthetic Construct
EVQLLESGGGLVQPGGSLRLSCAASGFTFSSYPMSWVRQAPGKGLEWVSAALGSGGSTYYADSVKGRFTISRDNSKNTLYLQMNSLRAEDTAVYYCARYWPMSLWGQGTLVTVSS

SEQ ID NO: 128 - protein, 108 aa, synthetic construct
  REGION 1..108: note = Synthetic Construct
EIVLTQSPGTLSLSPGERATLSCRASQSVSVRYLAWYQQKPGQAPRLLMYDASIRATGIPDRFSGSGSGTDFTLTISRLEPEDFAVYYCQQYGSWPITFGQGTKVEIK

SEQ ID NO: 129 - protein, 5 aa, synthetic construct
  REGION 1..5: note = Synthetic Construct
SYAMT

SEQ ID NO: 130 - protein, 7 aa, synthetic construct
  REGION 1..7: note = Synthetic Construct
GFTFGSY

SEQ ID NO: 131 - protein, 10 aa, synthetic construct
  REGION 1..10: note = Synthetic Construct
GFTFGSYAMT

SEQ ID NO: 132 - protein, 17 aa, synthetic construct
  REGION 1..17: note = Synthetic Construct
AISGSGGNTFYADSVKG

SEQ ID NO: 133 - protein, 6 aa, synthetic construct
  REGION 1..6: note = Synthetic Construct
SGSGGN

SEQ ID NO: 134 - protein, 10 aa, synthetic construct
  REGION 1..10: note = Synthetic Construct
VSPIASGMDY

SEQ ID NO: 135 - protein, 10 aa, synthetic construct
  REGION 1..10: note = Synthetic Construct
VSPIAAQMDY

SEQ ID NO: 136 - protein, 10 aa, synthetic construct
  REGION 1..10: note = Synthetic Construct
VSPIAALMDY

SEQ ID NO: 137 - protein, 10 aa, synthetic construct
  REGION 1..10: note = Synthetic Construct
VSPIAAPMDY

SEQ ID NO: 138 - protein, 17 aa, synthetic construct
  REGION 1..17: note = Synthetic Construct
AISGSGGNTFYADQRKG

SEQ ID NO: 139 - protein, 17 aa, synthetic construct
  REGION 1..17: note = Synthetic Construct
AIDYSGGNTFYADSVKG

SEQ ID NO: 140 - protein, 6 aa, synthetic construct
  REGION 1..6: note = Synthetic Construct
DYSSGN

SEQ ID NO: 141 - protein, 17 aa, synthetic construct
  REGION 1..17: note = Synthetic Construct
AISYQGGNTFYADSVKG

SEQ ID NO: 142 - protein, 6 aa, synthetic construct
  REGION 1..6: note = Synthetic Construct
SYQGGN

SEQ ID NO: 143 - protein, 17 aa, synthetic construct
  REGION 1..17: note = Synthetic Construct
AISLTGGNTFYADSVKG

SEQ ID NO: 144 - protein, 6 aa, synthetic construct
  REGION 1..6: note = Synthetic Construct
SLTGGN

SEQ ID NO: 145 - protein, 17 aa, synthetic construct
  REGION 1..17: note = Synthetic Construct
AISHAGGNTFYADSVKG

SEQ ID NO: 146 - protein, 6 aa, synthetic construct
  REGION 1..6: note = Synthetic Construct
SHAGGN

SEQ ID NO: 147 - protein, 17 aa, synthetic construct
  REGION 1..17: note = Synthetic Construct
AISGSGGNTFYADQLKG

SEQ ID NO: 148 - protein, 10 aa, synthetic construct
  REGION 1..10: note = Synthetic Construct
VSPIYAGMDY

SEQ ID NO: 149 - protein, 10 aa, synthetic construct
  REGION 1..10: note = Synthetic Construct
VSPIAAEMDY

SEQ ID NO: 150 - protein, 5 aa, synthetic construct
  REGION 1..5: note = Synthetic Construct
SYAMN

SEQ ID NO: 151 - protein, 7 aa, synthetic construct
  REGION 1..7: note = Synthetic Construct
GFTFSSY

SEQ ID NO: 152 - protein, 10 aa, synthetic construct
  REGION 1..10: note = Synthetic Construct
GFTFSSYAMN

SEQ ID NO: 153 - protein, 17 aa, synthetic construct
  REGION 1..17: note = Synthetic Construct
AISDSGGSTYYADSVKG

SEQ ID NO: 154 - protein, 6 aa, synthetic construct
  REGION 1..6: note = Synthetic Construct
SDSGGS

SEQ ID NO: 155 - protein, 6 aa, synthetic construct
  REGION 1..6: note = Synthetic Construct
YWPMDI

SEQ ID NO: 156 - protein, 5 aa, synthetic construct
  REGION 1..5: note = Synthetic Construct
SYPMS

SEQ ID NO: 157 - protein, 10 aa, synthetic construct
  REGION 1..10: note = Synthetic Construct
GFTFSSYPMS

SEQ ID NO: 158 - protein, 17 aa, synthetic construct
  REGION 1..17: note = Synthetic Construct
AIGGSGGSLPYADSVKG

SEQ ID NO: 159 - protein, 6 aa, synthetic construct
  REGION 1..6: note = Synthetic Construct
GGSGGS

SEQ ID NO: 160 - protein, 17 aa, synthetic construct
  REGION 1..17: note = Synthetic Construct
AILDSGGSTYYADSVKG

SEQ ID NO: 161 - protein, 6 aa, synthetic construct
  REGION 1..6: note = Synthetic Construct
YWPMDS

SEQ ID NO: 162 - protein, 17 aa, synthetic construct
  REGION 1..17: note = Synthetic Construct
AIGGSGGSTYYADSVKG

SEQ ID NO: 163 - protein, 17 aa, synthetic construct
  REGION 1..17: note = Synthetic Construct
AISDSGGSAWYADSVKG

SEQ ID NO: 164 - protein, 6 aa, synthetic construct
  REGION 1..6: note = Synthetic Construct
YWPMSL

SEQ ID NO: 165 - protein, 17 aa, synthetic construct
  REGION 1..17: note = Synthetic Construct
AISDFGGSTYYADSVKG

SEQ ID NO: 166 - protein, 6 aa, synthetic construct
  REGION 1..6: note = Synthetic Construct
SDFGGS

SEQ ID NO: 167 - protein, 17 aa, synthetic construct
  REGION 1..17: note = Synthetic Construct
AITASGGSTYYADSVKG

SEQ ID NO: 168 - protein, 6 aa, synthetic construct
  REGION 1..6: note = Synthetic Construct
TASGGS

SEQ ID NO: 169 - protein, 17 aa, synthetic construct
  REGION 1..17: note = Synthetic Construct
AISDSGGSRWYADSVKG

SEQ ID NO: 170 - protein, 6 aa, synthetic construct
  REGION 1..6: note = Synthetic Construct
YWPMTP

SEQ ID NO: 171 - protein, 17 aa, synthetic construct
  REGION 1..17: note = Synthetic Construct
AVLDSGGSTYYADSVKG

SEQ ID NO: 172 - protein, 6 aa, synthetic construct
  REGION 1..6: note = Synthetic Construct
LDSGGS

SEQ ID NO: 173 - protein, 6 aa, synthetic construct
  REGION 1..6: note = Synthetic Construct
YWPMSD

SEQ ID NO: 174 - protein, 17 aa, synthetic construct
  REGION 1..17: note = Synthetic Construct
AISDSGGSKWYADSVKG

SEQ ID NO: 175 - protein, 17 aa, synthetic construct
  REGION 1..17: note = Synthetic Construct
AISDSGGSGWYADSVKG

SEQ ID NO: 176 - protein, 17 aa, synthetic construct
  REGION 1..17: note = Synthetic Construct
AISDSGGSCWYADSVKG

SEQ ID NO: 177 - protein, 17 aa, synthetic construct
  REGION 1..17: note = Synthetic Construct
AIFASGGSTYYADSVKG

SEQ ID NO: 178 - protein, 6 aa, synthetic construct
  REGION 1..6: note = Synthetic Construct
FASGGS

SEQ ID NO: 179 - protein, 6 aa, synthetic construct
  REGION 1..6: note = Synthetic Construct
SGWGGS

SEQ ID NO: 180 - protein, 17 aa, synthetic construct
  REGION 1..17: note = Synthetic Construct
AIMSSGGPLYYADSVKG

SEQ ID NO: 181 - protein, 6 aa, synthetic construct
  REGION 1..6: note = Synthetic Construct
MSSGGP

SEQ ID NO: 182 - protein, 6 aa, synthetic construct
  REGION 1..6: note = Synthetic Construct
YWPMAL

SEQ ID NO: 183 - protein, 17 aa, synthetic construct
  REGION 1..17: note = Synthetic Construct
AILMSGGSTYYADSVKG

SEQ ID NO: 184 - protein, 6 aa, synthetic construct
  REGION 1..6: note = Synthetic Construct
LMSGGS

SEQ ID NO: 185 - protein, 17 aa, synthetic construct
  REGION 1..17: note = Synthetic Construct
AISDSGGYRYYADSVKG

SEQ ID NO: 186 - protein, 6 aa, synthetic construct
  REGION 1..6: note = Synthetic Construct
SDSGGY

SEQ ID NO: 187 - protein, 17 aa, synthetic construct
  REGION 1..17: note = Synthetic Construct
AILSSGGSTYYADSVKG

SEQ ID NO: 188 - protein, 6 aa, synthetic construct
  REGION 1..6: note = Synthetic Construct
LSSGGS

SEQ ID NO: 189 - protein, 6 aa, synthetic construct
  REGION 1..6: note = Synthetic Construct
YWPMSP

SEQ ID NO: 190 - protein, 17 aa, synthetic construct
  REGION 1..17: note = Synthetic Construct
AIGGSGGWSYYADSVKG

SEQ ID NO: 191 - protein, 6 aa, synthetic construct
  REGION 1..6: note = Synthetic Construct
GGSGGW

SEQ ID NO: 192 - protein, 17 aa, synthetic construct
  REGION 1..17: note = Synthetic Construct
ATVGSGGSIGYADSVKG

SEQ ID NO: 193 - protein, 6 aa, synthetic construct
  REGION 1..6: note = Synthetic Construct
VGSGGS

SEQ ID NO: 194 - protein, 17 aa, synthetic construct
  REGION 1..17: note = Synthetic Construct
AIGGSGGSIHYADSVKG

SEQ ID NO: 195 - protein, 17 aa, synthetic construct
  REGION 1..17: note = Synthetic Construct
AHIGSGGSTYYADSVKG

SEQ ID NO: 196 - protein, 6 aa, synthetic construct
  REGION 1..6: note = Synthetic Construct
IGSGGS

SEQ ID NO: 197 - protein, 6 aa, synthetic construct
  REGION 1..6: note = Synthetic Construct
YWPMDP

SEQ ID NO: 198 - protein, 17 aa, synthetic construct
  REGION 1..17: note = Synthetic Construct
AIGGSGGSLGYADSVKG

SEQ ID NO: 199 - protein, 17 aa, synthetic construct
  REGION 1..17: note = Synthetic Construct
AIGGSGTWTYYADSVKG

SEQ ID NO: 200 - protein, 6 aa, synthetic construct
  REGION 1..6: note = Synthetic Construct
GGSGTW

SEQ ID NO: 201 - protein, 17 aa, synthetic construct
  REGION 1..17: note = Synthetic Construct
ALFGSGGSTYYADSVKG

SEQ ID NO: 202 - protein, 6 aa, synthetic construct
  REGION 1..6: note = Synthetic Construct
FGSGGS

SEQ ID NO: 203 - protein, 17 aa, synthetic construct
  REGION 1..17: note = Synthetic Construct
AALGSGGSTYYADSVKG

SEQ ID NO: 204 - protein, 6 aa, synthetic construct
  REGION 1..6: note = Synthetic Construct
LGSGGS

SEQ ID NO: 205 - protein, 6 aa, synthetic construct
  REGION 1..6: note = Synthetic Construct
YWPMAD

SEQ ID NO: 206 - protein, 17 aa, synthetic construct
  REGION 1..17: note = Synthetic Construct
AISDSGGFVYYADSVKG

SEQ ID NO: 207 - protein, 6 aa, synthetic construct
  REGION 1..6: note = Synthetic Construct
SDSGGF

SEQ ID NO: 208 - protein, 17 aa, synthetic construct
  REGION 1..17: note = Synthetic Construct
ACLDSGGSTYYADSVKG

SEQ ID NO: 209 - protein, 12 aa, synthetic construct
  REGION 1..12: note = Synthetic Construct
RASQSVSSSYLA

SEQ ID NO: 210 - protein, 7 aa, synthetic construct
  REGION 1..7: note = Synthetic Construct
GASSRAT

SEQ ID NO: 211 - protein, 10 aa, synthetic construct
  REGION 1..10: note = Synthetic Construct
QHYGSPPSFT

SEQ ID NO: 212 - protein, 12 aa, synthetic construct
  REGION 1..12: note = Synthetic Construct
RASQSLGSFYLA

SEQ ID NO: 213 - protein, 10 aa, synthetic construct
  REGION 1..10: note = Synthetic Construct
KHYGWPPSFT

SEQ ID NO: 214 - protein, 10 aa, synthetic construct
  REGION 1..10: note = Synthetic Construct
QHYNYPPSFT

SEQ ID NO: 215 - protein, 12 aa, synthetic construct
  REGION 1..12: note = Synthetic Construct
RASQSVGDFYLA

SEQ ID NO: 216 - protein, 10 aa, synthetic construct
  REGION 1..10: note = Synthetic Construct
QHYPYPPSFT

SEQ ID NO: 217 - protein, 12 aa, synthetic construct
  REGION 1..12: note = Synthetic Construct
RASQSVSSSYPS

SEQ ID NO: 218 - protein, 12 aa, synthetic construct
  REGION 1..12: note = Synthetic Construct
RASQSVSAHYLA

SEQ ID NO: 219 - protein, 12 aa, synthetic construct
  REGION 1..12: note = Synthetic Construct
RASQSVSSFFLA

SEQ ID NO: 220 - protein, 10 aa, synthetic construct
  REGION 1..10: note = Synthetic Construct
KYYPYPPSFT

SEQ ID NO: 221 - protein, 7 aa, synthetic construct
  REGION 1..7: note = Synthetic Construct
DASIRAT

SEQ ID NO: 222 - protein, 9 aa, synthetic construct
  REGION 1..9: note = Synthetic Construct
QQYGSWPLT

SEQ ID NO: 223 - protein, 12 aa, synthetic construct
  REGION 1..12: note = Synthetic Construct
RASQSVSVLYLA

SEQ ID NO: 224 - protein, 9 aa, synthetic construct
  REGION 1..9: note = Synthetic Construct
QQYQRWPLT

SEQ ID NO: 225 - protein, 9 aa, synthetic construct
  REGION 1..9: note = Synthetic Construct
QQYQSWPLT

SEQ ID NO: 226 - protein, 12 aa, synthetic construct
  REGION 1..12: note = Synthetic Construct
RASQSVSDLYLA

SEQ ID NO: 227 - protein, 9 aa, synthetic construct
  REGION 1..9: note = Synthetic Construct
QQYQTWPLT

SEQ ID NO: 228 - protein, 12 aa, synthetic construct
  REGION 1..12: note = Synthetic Construct
RASQSVSNLYLA

SEQ ID NO: 229 - protein, 9 aa, synthetic construct
  REGION 1..9: note = Synthetic Construct
QQYQGWPLT

SEQ ID NO: 230 - protein, 12 aa, synthetic construct
  REGION 1..12: note = Synthetic Construct
RASQSVSAYYLA

SEQ ID NO: 231 - protein, 9 aa, synthetic construct
  REGION 1..9: note = Synthetic Construct
QQYERWPLT

SEQ ID NO: 232 - protein, 12 aa, synthetic construct
  REGION 1..12: note = Synthetic Construct
RASQSVSSLYLA

SEQ ID NO: 233 - protein, 9 aa, synthetic construct
  REGION 1..9: note = Synthetic Construct
QQYQVWPLT

SEQ ID NO: 234 - protein, 9 aa, synthetic construct
  REGION 1..9: note = Synthetic Construct
QQYLDWPLT

SEQ ID NO: 235 - protein, 12 aa, synthetic construct
  REGION 1..12: note = Synthetic Construct
RASQSVSALYLA

SEQ ID NO: 236 - protein, 9 aa, synthetic construct
  REGION 1..9: note = Synthetic Construct
QQYLAWPLT

SEQ ID NO: 237 - protein, 9 aa, synthetic construct
  REGION 1..9: note = Synthetic Construct
QQYFTWPLT

SEQ ID NO: 238 - protein, 12 aa, synthetic construct
  REGION 1..12: note = Synthetic Construct
RASQSVSPYYLA

SEQ ID NO: 239 - protein, 12 aa, synthetic construct
  REGION 1..12: note = Synthetic Construct
RASQSVSVEYLA

SEQ ID NO: 240 - protein, 9 aa, synthetic construct
  REGION 1..9: note = Synthetic Construct
QQYARWPLT

SEQ ID NO: 241 - protein, 12 aa, synthetic construct
  REGION 1..12: note = Synthetic Construct
RASQSVSELYLA

SEQ ID NO: 242 - protein, 9 aa, synthetic construct
  REGION 1..9: note = Synthetic Construct
QQYFGWPLT

SEQ ID NO: 243 - protein, 12 aa, synthetic construct
  REGION 1..12: note = Synthetic Construct
RASQSVEMSYLA

SEQ ID NO: 244 - protein, 9 aa, synthetic construct
  REGION 1..9: note = Synthetic Construct
QQYAHWPLT

SEQ ID NO: 245 - protein, 12 aa, synthetic construct
  REGION 1..12: note = Synthetic Construct
RASQSVSAQYLA

SEQ ID NO: 246 - protein, 12 aa, synthetic construct
  REGION 1..12: note = Synthetic Construct
GPSQSVSSSYLA

SEQ ID NO: 247 - protein, 12 aa, synthetic construct
  REGION 1..12: note = Synthetic Construct
RASQSVSSSYWA

SEQ ID NO: 248 - protein, 9 aa, synthetic construct
  REGION 1..9: note = Synthetic Construct
QQYESWPLT

SEQ ID NO: 249 - protein, 12 aa, synthetic construct
  REGION 1..12: note = Synthetic Construct
RGGQSVSSSYLA

SEQ ID NO: 250 - protein, 12 aa, synthetic construct
  REGION 1..12: note = Synthetic Construct
RASQSVSFLYLA

SEQ ID NO: 251 - protein, 12 aa, synthetic construct
  REGION 1..12: note = Synthetic Construct
RASQSVSSTYLA

SEQ ID NO: 252 - protein, 7 aa, synthetic construct
  REGION 1..7: note = Synthetic Construct
DASSRAP

SEQ ID NO: 253 - protein, 9 aa, synthetic construct
  REGION 1..9: note = Synthetic Construct
QQYSTSPLT

SEQ ID NO: 254 - protein, 12 aa, synthetic construct
  REGION 1..12: note = Synthetic Construct
RASQSVSPEYLA

SEQ ID NO: 255 - protein, 9 aa, synthetic construct
  REGION 1..9: note = Synthetic Construct
QQYSVWPLT

SEQ ID NO: 256 - protein, 9 aa, synthetic construct
  REGION 1..9: note = Synthetic Construct
QQYSAWPLT

SEQ ID NO: 257 - protein, 12 aa, synthetic construct
  REGION 1..12: note = Synthetic Construct
RASQSVSSVYLA

SEQ ID NO: 258 - protein, 9 aa, synthetic construct
  REGION 1..9: note = Synthetic Construct
QQYSTWPLT

SEQ ID NO: 259 - protein, 9 aa, synthetic construct
  REGION 1..9: note = Synthetic Construct
QQYSRWPLT

SEQ ID NO: 260 - protein, 12 aa, synthetic construct
  REGION 1..12: note = Synthetic Construct
RASQSVSPLYLA

SEQ ID NO: 261 - protein, 9 aa, synthetic construct
  REGION 1..9: note = Synthetic Construct
QQYSAFPLT

SEQ ID NO: 262 - protein, 12 aa, synthetic construct
  REGION 1..12: note = Synthetic Construct
WLSQSVSSTYLA

SEQ ID NO: 263 - protein, 9 aa, synthetic construct
  REGION 1..9: note = Synthetic Construct
QQYSEWPLT

SEQ ID NO: 264 - protein, 9 aa, synthetic construct
  REGION 1..9: note = Synthetic Construct
QQYSSWPLT

SEQ ID NO: 265 - protein, 12 aa, synthetic construct
  REGION 1..12: note = Synthetic Construct
RASQSVSSLFLA

SEQ ID NO: 266 - protein, 12 aa, synthetic construct
  REGION 1..12: note = Synthetic Construct
ACSQSVSSTYLA

SEQ ID NO: 267 - protein, 12 aa, synthetic construct
  REGION 1..12: note = Synthetic Construct
RASCDVSSTYLA

SEQ ID NO: 268 - protein, 9 aa, synthetic construct
  REGION 1..9: note = Synthetic Construct
QQYMRSPLT

SEQ ID NO: 269 - protein, 12 aa, synthetic construct
  REGION 1..12: note = Synthetic Construct
RASEAVPSTYLA

SEQ ID NO: 270 - protein, 12 aa, synthetic construct
  REGION 1..12: note = Synthetic Construct
CSSQSVSSTYLA

SEQ ID NO: 271 - protein, 12 aa, synthetic construct
  REGION 1..12: note = Synthetic Construct
RASVRVSSTYLA

SEQ ID NO: 272 - protein, 9 aa, synthetic construct
  REGION 1..9: note = Synthetic Construct
QQYMKWPLT

SEQ ID NO: 273 - protein, 12 aa, synthetic construct
  REGION 1..12: note = Synthetic Construct
RASQSVSAAYLA

SEQ ID NO: 274 - protein, 9 aa, synthetic construct
  REGION 1..9: note = Synthetic Construct
QQYMCWPLT

SEQ ID NO: 275 - protein, 12 aa, synthetic construct
  REGION 1..12: note = Synthetic Construct
RASQSVSSSYWG

SEQ ID NO: 276 - protein, 9 aa, synthetic construct
  REGION 1..9: note = Synthetic Construct
QQYQCWPLT

SEQ ID NO: 277 - protein, 12 aa, synthetic construct
  REGION 1..12: note = Synthetic Construct
RASQSVSSPYLA

SEQ ID NO: 278 - protein, 9 aa, synthetic construct
  REGION 1..9: note = Synthetic Construct
QQYKAWPLT

SEQ ID NO: 279 - protein, 12 aa, synthetic construct
  REGION 1..12: note = Synthetic Construct
RASQSVSYLYLA

SEQ ID NO: 280 - protein, 9 aa, synthetic construct
  REGION 1..9: note = Synthetic Construct
QQYMEWPLT

SEQ ID NO: 281 - protein, 9 aa, synthetic construct
  REGION 1..9: note = Synthetic Construct
QQYQAWPLT

SEQ ID NO: 282 - protein, 9 aa, synthetic construct
  REGION 1..9: note = Synthetic Construct
QQYQKWPLT

SEQ ID NO: 283 - protein, 12 aa, synthetic construct
  REGION 1..12: note = Synthetic Construct
RASQSVSAVYLA

SEQ ID NO: 284 - protein, 9 aa, synthetic construct
  REGION 1..9: note = Synthetic Construct
QQYRAWPLT

SEQ ID NO: 285 - protein, 12 aa, synthetic construct
  REGION 1..12: note = Synthetic Construct
RASIAVSSTYLA

SEQ ID NO: 286 - protein, 9 aa, synthetic construct
  REGION 1..9: note = Synthetic Construct
QQYMVWPLT

SEQ ID NO: 287 - protein, 12 aa, synthetic construct
  REGION 1..12: note = Synthetic Construct
RPRQSVSSSYLA

SEQ ID NO: 288 - protein, 9 aa, synthetic construct
  REGION 1..9: note = Synthetic Construct
QQYQDWPLT

SEQ ID NO: 289 - protein, 9 aa, synthetic construct
  REGION 1..9: note = Synthetic Construct
QQYQEWPLT

SEQ ID NO: 290 - protein, 12 aa, synthetic construct
  REGION 1..12: note = Synthetic Construct
RASQSVSASYLA

SEQ ID NO: 291 - protein, 9 aa, synthetic construct
  REGION 1..9: note = Synthetic Construct
QQYMSWPLT

SEQ ID NO: 292 - protein, 12 aa, synthetic construct
  REGION 1..12: note = Synthetic Construct
RASQSVSYMYLA

SEQ ID NO: 293 - protein, 9 aa, synthetic construct
  REGION 1..9: note = Synthetic Construct
QQYKSWPLT

SEQ ID NO: 294 - protein, 9 aa, synthetic construct
  REGION 1..9: note = Synthetic Construct
QQYYGWPLT

SEQ ID NO: 295 - protein, 12 aa, synthetic construct
  REGION 1..12: note = Synthetic Construct
RASQPISSSYLA

SEQ ID NO: 296 - protein, 9 aa, synthetic construct
  REGION 1..9: note = Synthetic Construct
QQYEFWPLT

SEQ ID NO: 297 - protein, 12 aa, synthetic construct
  REGION 1..12: note = Synthetic Construct
RASQGISSTYLA

SEQ ID NO: 298 - protein, 9 aa, synthetic construct
  REGION 1..9: note = Synthetic Construct
QQYAYWPLT

SEQ ID NO: 299 - protein, 12 aa, synthetic construct
  REGION 1..12: note = Synthetic Construct
RASQSVSVRYLA

SEQ ID NO: 300 - protein, 9 aa, synthetic construct
  REGION 1..9: note = Synthetic Construct
QQYGSWPIT

SEQ ID NO: 301 - skipped

SEQ ID NO: 302 - protein, 7 aa, synthetic construct
  REGION 1..7: note = Synthetic Construct
  SITE 5: note = MISC_FEATURE - Xaa is G or S
GFTFXSY

SEQ ID NO: 303 - protein, 10 aa, synthetic construct
  REGION 1..10: note = Synthetic Construct
  SITE 5: note = MISC_FEATURE - Xaa is G or S
  SITE 8: note = MISC_FEATURE - Xaa is A or P
  SITE 10: note = MISC_FEATURE - Xaa is T, N, or S
GFTFXSYXMX

SEQ ID NO: 304 - protein, 17 aa, synthetic construct
  REGION 1..17: note = Synthetic Construct
AISGWGGSLPYADSVKG

SEQ ID NO: 305 - protein, 17 aa, synthetic construct
  REGION 1..17: note = Synthetic Construct
  SITE 2: note = MISC_FEATURE - Xaa is I, V, T, H, L, A, or C
  SITE 3: note = MISC_FEATURE - Xaa is S, D, G, T, I, L, F, M, or V
  SITE 4: note = MISC_FEATURE - Xaa is G, Y, L, H, D, A, S, or M
  SITE 5: note = MISC_FEATURE - Xaa is S, Q, T, A, F, or W
  SITE 7: note = MISC_FEATURE - Xaa is G or T
  SITE 8: note = MISC_FEATURE - Xaa is N, S, P, Y, W, or F
  SITE 9: note = MISC_FEATURE - Xaa is S, T, I, L, T, A, R, V, K, G, or C
  SITE 10: note = MISC_FEATURE - Xaa is F, Y, P, W, H, or G
  SITE 14: note = MISC_FEATURE - Xaa is V, R, or L
  SITE 15: note = MISC_FEATURE - Xaa is G or T
AXXXXGXXXXYADXXKG

SEQ ID NO: 306 - skipped

SEQ ID NO: 307 - protein, 10 aa, synthetic construct
  REGION 1..10: note = Synthetic Construct
  SITE 5: note = MISC_FEATURE - Xaa is A or Y
  SITE 6: note = MISC_FEATURE - Xaa is A or S
  SITE 7: note = MISC_FEATURE - Xaa is G, Q, L, P, or E
VSPIXXXMDY

SEQ ID NO: 308 - protein, 6 aa, synthetic construct
  REGION 1..6: note = Synthetic Construct
  SITE 5: note = MISC_FEATURE - Xaa is D, S, T, or A
  SITE 6: note = MISC_FEATURE - Xaa is I, S, L, P, or D
YWPMXX

SEQ ID NO: 309 - skipped

SEQ ID NO: 310 - protein, 7 aa, synthetic construct
  REGION 1..7: note = Synthetic Construct
  SITE 1: note = MISC_FEATURE - Xaa is G or D
  SITE 4: note = MISC_FEATURE - Xaa is S or I
  SITE 7: note = MISC_FEATURE - Xaa is T or P
XASXRAX

SEQ ID NO: 311 - protein, 10 aa, synthetic construct
  REGION 1..10: note = Synthetic Construct
  SITE 1: note = MISC_FEATURE - Xaa is Q or K
  SITE 2: note = MISC_FEATURE - Xaa is H or Y
  SITE 4: note = MISC_FEATURE - Xaa is G, N, or P
  SITE 5: note = MISC_FEATURE - Xaa is S, W, or Y
XXYXXPPSFT

SEQ ID NO: 312 - protein, 9 aa, synthetic construct
  REGION 1..9: note = Synthetic Construct
  SITE 4: note = MISC_FEATURE - Xaa is G, Q, E, L, F, A, S, M, K, R, or Y
  SITE 5: note = MISC_FEATURE - Xaa is S, R, T, G, V, F, Y, D, A, H, V, E, K, or C
  SITE 6: note = MISC_FEATURE - Xaa is W, F, or S
  SITE 8: note = MISC_FEATURE - Xaa is L or I
QQYXXXPXT

SEQ ID NO: 313 - protein, 119 aa, synthetic construct
  REGION 1..119: note = Synthetic Construct
  SITE 30: note = MISC_FEATURE - Xaa is G or S
  SITE 33: note = MISC_FEATURE - Xaa is A or P
  SITE 35: note = MISC_FEATURE - Xaa is T, N, or S
  SITE 51: note = MISC_FEATURE - Xaa is I, V, T, H, L, A, or C
  SITE 52: note = MISC_FEATURE - Xaa is S, D, G, T, I, L, F, M, or V
  SITE 53: note = MISC_FEATURE - Xaa is G, Y, L, H, D, A, S, or M
  SITE 54: note = MISC_FEATURE - Xaa is S, Q, T, A, F, or W
  SITE 56: note = MISC_FEATURE - Xaa is G or T
  SITE 57: note = MISC_FEATURE - Xaa is N, S, P, Y, W, or F
  SITE 58: note = MISC_FEATURE - Xaa is S, T, I, L, T, A, R, V, K, G, or C
  SITE 59: note = MISC_FEATURE - Xaa is F, Y, P, W, H, or G
  SITE 63: note = MISC_FEATURE - Xaa is V, R, or L
  SITE 64: note = MISC_FEATURE - Xaa is G or T
  SITE 103: note = MISC_FEATURE - Xaa is A or Y
  SITE 104: note = MISC_FEATURE - Xaa is A or S
  SITE 105: note = MISC_FEATURE - Xaa is G, Q, L, P, or E
EVQLLESGGGLVQPGGSLRLSCAASGFTFXSYXMXWVRQAPGKGLEWVSAXXXXGXXXXYADXXKGRFTISRDNSKNTLYLQMNSLRAEDTAVYYCARVSPIXXXMDYWGQGTLVTVSS

SEQ ID NO: 314 - protein, 115 aa, synthetic construct
  REGION 1..115: note = Synthetic Construct
  SITE 30: note = MISC_FEATURE - Xaa is G or S
  SITE 33: note = MISC_FEATURE - Xaa is A or P
  SITE 35: note = MISC_FEATURE - Xaa is T, N, or S
  SITE 51: note = MISC_FEATURE - Xaa is I, V, T, H, L, A, or C
  SITE 52: note = MISC_FEATURE - Xaa is S, D, G, T, I, L, F, M, or V
  SITE 53: note = MISC_FEATURE - Xaa is G, Y, L, H, D, A, S, or M
  SITE 54: note = MISC_FEATURE - Xaa is S, Q, T, A, F, or W
  SITE 56: note = MISC_FEATURE - Xaa is G or T
  SITE 57: note = MISC_FEATURE - Xaa is N, S, P, Y, W, or F
  SITE 58: note = MISC_FEATURE - Xaa is S, T, I, L, T, A, R, V, K, G, or C
  SITE 59: note = MISC_FEATURE - Xaa is F, Y, P, W, H, or G
  SITE 63: note = MISC_FEATURE - Xaa is V, R, or L
  SITE 64: note = MISC_FEATURE - Xaa is G or T
  SITE 103: note = MISC_FEATURE - Xaa is D, S, T, or A
  SITE 104: note = MISC_FEATURE - Xaa is I, S, L, P, or D
EVQLLESGGGLVQPGGSLRLSCAASGFTFXSYXMXWVRQAPGKGLEWVSAXXXXGXXXXYADXXKGRFTISRDNSKNTLYLQMNSLRAEDTAVYYCARYWPMXXWGQGTLVTVSS

SEQ ID NO: 315 - protein, 109 aa, synthetic construct
  REGION 1..109: note = Synthetic Construct
  SITE 24: note = MISC_FEATURE - Xaa is R, G, W, A, or C
  SITE 25: note = MISC_FEATURE - Xaa is A, P, G, L, C, or S
  SITE 26: note = MISC_FEATURE - Xaa is S, G, or R
  SITE 27: note = MISC_FEATURE - Xaa is Q, C, E, V, or I
  SITE 28: note = MISC_FEATURE - Xaa is S, P, G, A, R, or D
  SITE 29: note = MISC_FEATURE - Xaa is V, G, I, or L
  SITE 30: note = MISC_FEATURE - Xaa is S, E, D, P, or G
  SITE 31: note = MISC_FEATURE - Xaa is S, P, F, A, M, E, V, N, D, or Y
  SITE 32: note = MISC_FEATURE - Xaa is I, T, V, E, S, A, M, Q, Y, H, R, or F
  SITE 33: note = MISC_FEATURE - Xaa is Y or F
  SITE 34: note = MISC_FEATURE - Xaa is L, W, or P
  SITE 35: note = MISC_FEATURE - Xaa is A, S, or G
  SITE 51: note = MISC_FEATURE - Xaa is G or D
  SITE 54: note = MISC_FEATURE - Xaa is S or I
  SITE 57: note = MISC_FEATURE - Xaa is T or P
  SITE 90: note = MISC_FEATURE - Xaa is Q or K
  SITE 91: note = MISC_FEATURE - Xaa is H or Y
  SITE 93: note = MISC_FEATURE - Xaa is G, N, or P
  SITE 94: note = MISC_FEATURE - Xaa is S, W, or Y
EIVLTQSPGTLSLSPGERATLSCXXXXXXXXXXXXWYQQKPGQAPRLLMYXASXRAXGIPDRFSGSGSGTDFTLTISRLEPEDFAVYYCXXYXXPPSFTFGQGTKVEIK

SEQ ID NO: 316 - protein, 107 aa, synthetic construct
  REGION 1..107: note = Synthetic Construct
  SITE 24: note = MISC_FEATURE - Xaa is R, G, W, A, or C
  SITE 25: note = MISC_FEATURE - Xaa is A, P, G, L, C, or S
  SITE 26: note = MISC_FEATURE - Xaa is S, G, or R
  SITE 27: note = MISC_FEATURE - Xaa is Q, C, E, V, or I
  SITE 28: note = MISC_FEATURE - Xaa is S, L, P, G, A, R, or D
  SITE 29: note = MISC_FEATURE - Xaa is V, G, or I
  SITE 30: note = MISC_FEATURE - Xaa is S, E, D, or P
  SITE 31: note = MISC_FEATURE - Xaa is S, P, F, A, M, E, V, N, D, or Y
  SITE 32: note = MISC_FEATURE - Xaa is I, T, V, E, S, A, M, Q, Y, H, or R
  SITE 33: note = MISC_FEATURE - Xaa is Y or F
  SITE 34: note = MISC_FEATURE - Xaa is L, W, or P
  SITE 35: note = MISC_FEATURE - Xaa is A, S, or G
  SITE 51: note = MISC_FEATURE - Xaa is G or D
  SITE 54: note = MISC_FEATURE - Xaa is S or I
  SITE 57: note = MISC_FEATURE - Xaa is T or P
  SITE 93: note = MISC_FEATURE - Xaa is G, Q, E, L, F, A, S, M, R, K, or Y
  SITE 94: note = MISC_FEATURE - Xaa is S, R, T, G, R, V, D, A, H, E, K, C, F, or Y
  SITE 95: note = MISC_FEATURE - Xaa is W, S, or F
  SITE 97: note = MISC_FEATURE - Xaa is L or I
EIVLTQSPGTLSLSPGERATLSCXXXXXXXXXXXXWYQQKPGQAPRLLMYXASXRAXGIPDRFSGSGSGTDFTLTISRLEPEDFAVYYCQQYXXXPXFGQGTKVEIK

SEQ ID NO: 317 - protein, 108 aa, synthetic construct
  REGION 1..108: note = Synthetic Construct
EIVLTQSPGTLSLSPGERATLSCRASQSVSALYLAWYQQKPGQAPRLLIYDASSRAPGIPDRFSGSGSGTDFTLTISRLEPEDFAVYYCQQYSAWPLTFGQGTKVEIK

SEQ ID NO: 318 - protein, 5 aa, synthetic construct
  REGION 1..5: note = Synthetic Construct
LLQGG

SEQ ID NO: 319 - protein, 112 aa, synthetic construct
  REGION 1..112: note = Synthetic Construct
DIVMTQSPDSLAVSLGERATINCTSSQSLFNVRSRKNYLAWYQQKPGQPPKLLISWASTRESGVPDRFSGSGSGTDFTLTISSLQAEDVAVYYCKQSYDLFTFGSGTKLEIK

SEQ ID NO: 320 - protein, 121 aa, synthetic construct
  REGION 1..121: note = Synthetic Construct
EVQLVESGGGLVQPGGSLRLSCAASGFTFSDYYMTWVRQAPGKGLEWVAFIRNRARGYTSDHNASVKGRFTISRDNAKNSLYLQMNSLRAEDTAVYYCARDRPSYYVLDYWGQGTTVTVSS

SEQ ID NO: 321 - protein, 112 aa, synthetic construct
  REGION 1..112: note = Synthetic Construct
DIVMTQSPDSLAVSLGERATINCKSSQSLFNVRSRKNYLAWYQQKPGQPPKLLISWASTRESGVPDRFSGSGSGTDFTLTISSLQAEDVAVYYCKQSYDLFTFGSGTKLEIK

SEQ ID NO: 322 - protein, 121 aa, synthetic construct; identical to SEQ ID NO: 320
  REGION 1..121: note = Synthetic Construct

SEQ ID NO: 323 - protein, 112 aa, synthetic construct; identical to SEQ ID NO: 321
  REGION 1..112: note = Synthetic Construct

SEQ ID NO: 324 - protein, 121 aa, synthetic construct
  REGION 1..121: note = Synthetic Construct
EVQLVESGGGLVQPGGSLRLSCAASGFTFSDYYMTWVRQAPGKGLEWVAFIRNRARGYTSDHNPSVKGRFTISRDNAKNSLYLQMNSLRAEDTAVYYCARDRPSYYVLDYWGQGTTVTVSS

SEQ ID NO: 325 - protein, 112 aa, synthetic construct; identical to SEQ ID NO: 321
  REGION 1..112: note = Synthetic Construct

SEQ ID NO: 326 - protein, 121 aa, synthetic construct
  REGION 1..121: note = Synthetic Construct
EVQLVESGGGLVQPGGSLRLSCAASGFTFSDYYMTWVRQAPGKGLEWVAFIRNRARGYTSDYAESVKGRFTISRDNAKNSLYLQMNSLRAEDTAVYYCARDRPSYYVLDYWGQGTTVTVSS

SEQ ID NO: 327 - protein, 112 aa, synthetic construct; identical to SEQ ID NO: 321
  REGION 1..112: note = Synthetic Construct

SEQ ID NO: 328 - protein, 121 aa, synthetic construct
  REGION 1..121: note = Synthetic Construct
EVQLVESGGGLVQPGGSLRLSCAASGFTFSDYYMTWVRQAPGKGLEWVAFIRNRARGYTSDYADSVKGRFTISRDNAKNSLYLQMNSLRAEDTAVYYCARDRPSYYVLDYWGQGTTVTVSS

SEQ ID NO: 329 - protein, 112 aa, synthetic construct; identical to SEQ ID NO: 319
  REGION 1..112: note = Synthetic Construct

SEQ ID NO: 330 - protein, 121 aa, synthetic construct
  REGION 1..121: note = Synthetic Construct
EVQLVESGGGLVQPGGSLRLSCAASGFTFSDYYMTWVRQAPGKGLEWVAFIRNRARGYTSDYAPSVKGRFTISRDNAKNSLYLQMNSLRAEDTAVYYCARDRPSYYVLDYWGQGTTVTVSS

SEQ ID NO: 331 - protein, 5 aa, synthetic construct
  REGION 1..5: note = Synthetic Construct
DYYMT

SEQ ID NO: 332 - protein, 7 aa, synthetic construct
  REGION 1..7: note = Synthetic Construct
GFTFSDY

SEQ ID NO: 333 - protein, 10 aa, synthetic construct
  REGION 1..10: note = Synthetic Construct
GFTFSDYYMT

SEQ ID NO: 334 - protein, 19 aa, synthetic construct
  REGION 1..19: note = Synthetic Construct
FIRNRARGYTSDHNASVKG

SEQ ID NO: 335 - protein, 10 aa, synthetic construct
  REGION 1..10: note = Synthetic Construct
DRPSYYVLDY

SEQ ID NO: 336 - protein, 19 aa, synthetic construct
  REGION 1..19: note = Synthetic Construct
FIRNRARGYTSDHNPSVKG

SEQ ID NO: 337 - protein, 19 aa, synthetic construct
  REGION 1..19: note = Synthetic Construct
FIRNRARGYTSDYAESVKG

SEQ ID NO: 338 - protein, 19 aa, synthetic construct
  REGION 1..19: note = Synthetic Construct
FIRNRARGYTSDYADSVKG

SEQ ID NO: 339 - protein, 19 aa, synthetic construct
  REGION 1..19: note = Synthetic Construct
FIRNRARGYTSDYAPSVKG

SEQ ID NO: 340 - protein, 17 aa, synthetic construct
  REGION 1..17: note = Synthetic Construct
TSSQSLFNVRSRKNYLA

SEQ ID NO: 341 - protein, 7 aa, synthetic construct
  REGION 1..7: note = Synthetic Construct
WASTRES

SEQ ID NO: 342 - protein, 8 aa, synthetic construct
  REGION 1..8: note = Synthetic Construct
KQSYDLFT

SEQ ID NO: 343 - protein, 17 aa, synthetic construct
  REGION 1..17: note = Synthetic Construct
KSSQSLFNVRSRKNYLA

SEQ ID NO: 344 - protein, 112 aa, synthetic construct
  REGION 1..112: note = Synthetic Construct
DIVMTQSPDSLAVSLGERATINCKSSQSLFNVRSRKNYLAWYQQKPGQPPKLLIYWASTRESGVPDRFSGSGSGTDFTLTISSLQAEDVAVYYCKQSYDLFTFGSGTKLEIK

SEQ ID NO: 345 - protein, 121 aa, synthetic construct; identical to SEQ ID NO: 324
  REGION 1..121: note = Synthetic Construct

SEQ ID NO: 346 - protein, 112 aa, synthetic construct
  REGION 1..112: note = Synthetic Construct
DIVMTQSPDSLAVSLGERATINCKSSQSLFNVRSRKNYLAWYQQKPGQPPKLLISWASTRESGVPDRFSGSGSGTDFTLTISSLQAEDVAVYYCKQSYDLFTFGQGTKLEIK

SEQ ID NO: 347 - protein, 121 aa, synthetic construct; identical to SEQ ID NO: 324
  REGION 1..121: note = Synthetic Construct

SEQ ID NO: 348 - protein, 112 aa, synthetic construct
  REGION 1..112: note = Synthetic Construct
DIVMTQSPDSLAVSLGERATINCKSSQSLFNVRSRKNYLAWYQQKPGQPPKLLIYWASTRESGVPDRFSGSGSGTDFTLTISSLQAEDVAVYYCKQSYDLFTFGQGTKLEIK

SEQ ID NO: 349 - protein, 121 aa, synthetic construct; identical to SEQ ID NO: 324
  REGION 1..121: note = Synthetic Construct

SEQ ID NO: 350 - protein, 112 aa, synthetic construct
  REGION 1..112: note = Synthetic Construct
DIVMSQSPPSLAVSVGDKVTMSCTSSQSLFNSRSRKNYLAWYQQKSGQSPKLLISWASTRESGVPDRFTGSGSGTDFTLTISSVQAEDLAVYYCKQSYDLFTFGSGTKLEIK

SEQ ID NO: 351 - protein, 121 aa, synthetic construct
  REGION 1..121: note = Synthetic Construct
EVKLVESGGGLVQPGGSLRLSCATFGFTFTDYYMTWVRQPPGKALEWVAFIRNRARGYTSDHNASVKGRFTISRDNSQNILYLQMNTLRAEDSATYYCARDRPSYYVLDYWGQGTTVTVSS

SEQ ID NO: 352 - protein, 112 aa, synthetic construct
  REGION 1..112: note = Synthetic Construct
DIVMSQSPSSLAVSAGEKVTMSCKSSQSLLNSRTRKNYLAWYQQKPGQSPKLLIYWASTRESGVPDRFTGSGSGTDFTLTIDSVQPEDLAVYYCTQSFILRTFGGGTKLEIK

SEQ ID NO: 353 - protein, 184 aa, Homo sapiens
MLQMAGQCSQNEYFDSLLHACIPCQLRCSSNTPPLTCQRYCNASVTNSVKGTNAILWTCLGLSLIISLAVFVLMFLLRKINSEPLKDEFKNTGSGLLGMANIDLEKSRTGDEIILPRGLEYTVEECTCEDCIKSKPKVDSDHCFPLPAMEEGATILVTTKTNDYCKSLPAALSATEIEKSISAR

SEQ ID NO: 354 - protein, 119 aa, synthetic construct
  REGION 1..119: note = Synthetic Construct
QVQLQQPGSELVRPGASVILSCKASGYTFTSYWMHWVRQRPGQGLEWIGNIYSGGDTINYDEKFKNKAILTVDTSSSTAYMHLSSLTSEDSAVYYCTRDATSRYFFDYWGQGTTVTVSS

SEQ ID NO: 355 - protein, 112 aa, synthetic construct
  REGION 1..112: note = Synthetic Construct
DIVMSQSPSSLAVSAGEKVTMSCKSSQSLLNSRTRKNYLAWYQQKPGQSPKLLIYWASTRASGVPDRFTGSGSGTDFTLTISSVQAEDLAIYYCKQSFILRTFGGGTKLEIK

SEQ ID NO: 356 - protein, 117 aa, synthetic construct
  REGION 1..117: note = Synthetic Construct
QVQLQQSGPDLVKPGASVEISCKASGYSFTTYYLHWVRQRPGQGLEWIGWIFPGSDNTKYNEKFKGKATLTADTSSSTAYMQLSSLTSEDSAVYFCARNRDYYFDYWGQGTTVTVSS

SEQ ID NO: 357 - protein, 215 aa, synthetic construct
  REGION 1..215: note = Synthetic Construct
EIVLTQSPGTLSLSPGERATLSCRASQSVSSSYLAWYQQKPGQAPRLLMYDASIRATGIPDRFSGSGSGTDFTLTISRLEPEDFAVYYCQQYQSWPLTFGQGTKVEIKRTVAAPSVFIFPPSDEQLKSGTASVVCLLNNFYPREAKVQWKVDNALQSGNSQESVTEQDSKDSTYSLSSTLTLSKADYEKHKVYACEVTHQGLSSPVTKSFNRGEC

SEQ ID NO: 358 - protein, 255 aa, synthetic construct
  REGION 1..255: note = Synthetic Construct
EVQLLESGGGLVQPGGSLRLSCAASGFTFSSYPMSWVRQAPGKGLEWVSAIGGSGGSLPYADSVKGRFTISRDNSKNTLYLQMNSLRAEDTAVYYCARYWPMDIWGQGTLVTVSSASTKGPSVFPLAPSSKSTSGGTAALGCLVKDYFPEPVTVSWNSGALTSGVHTFPAVLQSSGLYSLSSVVTVPSSSLGTQTYICNVNHKPSNTKVDKKVEPKSCDKTHTCPPCPAPELLGGPSVFLFPPKPKDTLMISRTP

SEQ ID NO: 359 - protein, 6 aa, synthetic construct
  REGION 1..6: note = Synthetic Construct
SGSGGS

SEQ ID NO: 360 - protein, 17 aa, synthetic construct
  REGION 1..17: note = Synthetic Construct
AISGSGGSTFYADSVKG

SEQ ID NO: 361 - protein, 9 aa, synthetic construct
  REGION 1..9: note = Synthetic Construct
VGTSGAFGI

SEQ ID NO: 362 - protein, 7 aa, synthetic construct
  REGION 1..7: note = Synthetic Construct
GASSRAY

SEQ ID NO: 363 - protein, 118 aa, synthetic construct
  REGION 1..118: note = Synthetic Construct
EVQLLESGGGLVQPGGSLRLSCAASGFTFSSYAMSWVRQAPGKGLEWVSAISASGGSTYYADSVKGRFTISRDNSKNTLYLQMNSLRAEDTAVYYCARLSWSGAFDNWGQGTLVTVSS

SEQ ID NO: 364 - protein, 109 aa, synthetic construct
  REGION 1..109: note = Synthetic Construct
EIVLTQSPGTLSLSPGERATLSCRASQNVSSSYLAWYQQKPGQAPRLLIYGASYRATGIPDRFSGSGSGTDFTLTISRLEPEDFAVYYCQHYGSPPSFTFGQGTKVEIK

SEQ ID NO: 365 - protein, 118 aa, synthetic construct
  REGION 1..118: note = Synthetic Construct
EVQLLESGGGLVQPGGSLRLSCAASGFTFRSYAMSWVRQAPGKGLEWVSAISGSGGSTFYADSVKGRFTISRDNSKNTLYLQMNSLRAEDTAVYYCATVGTSGAFGIWGQGTLVTVSS

SEQ ID NO: 366 - protein, 5 aa, synthetic construct
  REGION 1..5: note = Synthetic Construct
SYAMS

SEQ ID NO: 367 - protein, 10 aa, synthetic construct
  REGION 1..10: note = Synthetic Construct
GFTFSSYAMS

SEQ ID NO: 368 - protein, 6 aa, synthetic construct
  REGION 1..6: note = Synthetic Construct
SASGGS

SEQ ID NO: 369 - protein, 17 aa, synthetic construct
  REGION 1..17: note = Synthetic Construct
AISASGGSTYYADSVKG

SEQ ID NO: 370 - protein, 9 aa, synthetic construct
  REGION 1..9: note = Synthetic Construct
LSWSGAFDN

SEQ ID NO: 371 - protein, 7 aa, synthetic construct
  REGION 1..7: note = Synthetic Construct
GFTFRSY

SEQ ID NO: 372 - protein, 10 aa, synthetic construct
  REGION 1..10: note = Synthetic Construct
GFTFRSYAMS

SEQ ID NO: 373 - protein, 112 aa, synthetic construct; identical to SEQ ID NO: 352
  REGION 1..112: note = Synthetic Construct

SEQ ID NO: 374 - protein, 119 aa, synthetic construct; identical to SEQ ID NO: 354
  REGION 1..119: note = Synthetic Construct

SEQ ID NO: 375 - protein, 112 aa, synthetic construct; identical to SEQ ID NO: 355
  REGION 1..112: note = Synthetic Construct

SEQ ID NO: 376 - protein, 117 aa, synthetic construct; identical to SEQ ID NO: 356
  REGION 1..117: note = Synthetic Construct

SEQ ID NO: 377 - protein, 109 aa, synthetic construct
  REGION 1..109: note = Synthetic Construct
QAVVTQESALTTSPGEAVTLTCRSSTGAVTTSNYANWVQEKPDHLFTGLIGGTNTRAPGVPARFSGSLIGDKAALTITGAQTEDEAIYFCVLWYNNYWVFGGGTKLTVL

SEQ ID NO: 378 - protein, 124 aa, synthetic construct
  REGION 1..124: note = Synthetic Construct
EVQLVESGGGLVRPEGSLRLSCAASGFTFNTYAMNWVRQAPGKGLEWVGRIRSKINNYATYYAESVKGRFTLSRDDSLSMVYLQMNSLKNEDTAMYYCVRHETLRSGISWFASWGQGTLVTVSS

SEQ ID NO: 379 - protein, 109 aa, synthetic construct
  REGION 1..109: note = Synthetic Construct
QAVVTQESALTTSPGETVTLTCRSSTGAVTTSNYANWVQEKPDHLFTGLIGGTNNRAPGVPARFSGSLIGDKAALTITGAQTEDEAIYFCALWYSNHWVFGGGTKLTVL

SEQ ID NO: 380 - protein, 124 aa, synthetic construct
  REGION 1..124: note = Synthetic Construct
EVQLVDSGGGLVQPKGSLKLSCAASGFTFNTYAMNWVRQAPGKGLEWVARIRSKSNNYATYYADSVKDRFTISRDDSQSRLYLQMNNLKTEDTAMYYCVRHETLRSGISWFANWGQGTLVTVSS

SEQ ID NO: 381 - protein, 109 aa, synthetic construct
  REGION 1..109: note = Synthetic Construct
QAVVTQEPSLTVSPGGTVTLTCRSSTGAVTTSNYANWVQQKPGQAPRGLIGGTNTRAPGTPARFSGSLLGGKAALTLSGAQPEDEAEYYCVLWYNNYWVFGGGTKLTVL

SEQ ID NO: 382 - protein, 124 aa, synthetic construct
  REGION 1..124: note = Synthetic Construct
EVQLVESGGGLVKPGGSLRLSCAASGFTFSTYAMNWVRQAPGKGLEWVGRIRSKINNYATYYAESVKGRFTISRDDSKNTLYLQMNSLKTEDTAVYYCVRHETLRSGISWFASWGQGTLVTVSS

SEQ ID NO: 383 - protein, 109 aa, synthetic construct
  REGION 1..109: note = Synthetic Construct
QAVVTQEPSLTVSPGGTVTLTCRSSTGAVTTSNYANWVQQKPGQAPRGLIGGTNTRAPGTPARFSGSLLGGKAALTLSGAQPEDEAEYYCVLWYNNHWVFGGGTKLTVL

SEQ ID NO: 384 - protein, 124 aa, synthetic construct; identical to SEQ ID NO: 382
  REGION 1..124: note = Synthetic Construct

SEQ ID NO: 385 - protein, 109 aa, synthetic construct
  REGION 1..109: note = Synthetic Construct
QAVVTQEPSLTVSPGGTVTLTCRASTGAVTTSNYANWVQQKPGQAPRGLIGGTNTRAPGTPARFSGSLLGGKAALTLSGAQPEDEAEYYCVLWYNNHWVFGGGTKLTVL

SEQ ID NO: 386 - protein, 124 aa, synthetic construct; identical to SEQ ID NO: 382
  REGION 1..124: note = Synthetic Construct

SEQ ID NO: 387 - protein, 109 aa, synthetic construct
  REGION 1..109: note = Synthetic Construct
QAVVTQEPSLTVSPGGTVTLTCRTSTGAVTTSNYANWVQQKPGQAPRGLIGGTNTRAPGTPARFSGSLLGGKAALTLSGAQPEDEAEYYCVLWYNNHWVFGGGTKLTVL

SEQ ID NO: 388 - protein, 124 aa, synthetic construct; identical to SEQ ID NO: 382
  REGION 1..124: note = Synthetic Construct

SEQ ID NO: 389 - protein, 109 aa, synthetic construct; identical to SEQ ID NO: 381
  REGION 1..109: note = Synthetic Construct

SEQ ID NO: 390 - protein, 124 aa, synthetic construct
  REGION 1..124: note = Synthetic Construct
EVQLVESGGGLVKPGGSLRLSCAASGFTFNTYAMNWVRQAPGKGLEWVGRIRSKINNYATYYAESVKGRFTISRDDSKNTLYLQMNSLKTEDTAVYYCVRHETLRSGISWFASWGQGTLVTVSS

SEQ ID NO: 391 - protein, 109 aa, synthetic construct; identical to SEQ ID NO: 383
  REGION 1..109: note = Synthetic Construct

SEQ ID NO: 392 - protein, 124 aa, synthetic construct; identical to SEQ ID NO: 390
  REGION 1..124: note = Synthetic Construct

SEQ ID NO: 393 - protein, 109 aa, synthetic construct; identical to SEQ ID NO: 387
  REGION 1..109: note = Synthetic Construct

SEQ ID NO: 394 - protein, 124 aa, synthetic construct
  REGION 1..124: note = Synthetic Construct
EVQLVESGGGLVKPGGSLRLSCAASGFTFSTYAMNWVRQAPGKGLEWVGRIRSHINNYATYYAESVKGRFTISRDDSKNTLYLQMNSLKTEDTAVYYCVRHETLRSGISWFASWGQGTLVTVSS

SEQ ID NO: 395 - protein, 109 aa, synthetic construct; identical to SEQ ID NO: 387
  REGION 1..109: note = Synthetic Construct

SEQ ID NO: 396 - protein, 124 aa, synthetic construct
  REGION 1..124: note = Synthetic Construct
EVQLVESGGGLVKPGGSLRLSCAASGFTFSTYAMNWVRQAPGKGLEWVGRIRSKYNNYATYYAESVKGRFTISRDDSKNTLYLQMNSLKTEDTAVYYCVRHETLRSGISWFASWGQGTLVTVSS

SEQ ID NO: 397 - protein, 109 aa, synthetic construct; identical to SEQ ID NO: 387
  REGION 1..109: note = Synthetic Construct

SEQ ID NO: 398 - protein, 124 aa, synthetic construct
  REGION 1..124: note = Synthetic Construct
EVQLVESGGGLVKPGGSLRLSCAASGFTFSTYAMNWVRQAPGKGLEWVGRERSKINNYATYYAESVKGRFTISRDDSKNTLYLQMNSLKTEDTAVYYCVRHETLRSGISWFASWGQGTLVTVSS

SEQ ID NO: 399 - protein, 109 aa, synthetic construct; identical to SEQ ID NO: 387
  REGION 1..109: note = Synthetic Construct

SEQ ID NO: 400 - protein, 124 aa, synthetic construct
  REGION 1..124: note = Synthetic Construct
EVQLVESGGGLVKPGGSLRLSCAASGFTFSTYAMNWVRQAPGKGLEWVGRIRSKINNYKTYYAESVKGRFTISRDDSKNTLYLQMNSLKTEDTAVYYCVRHETLRSGISWFASWGQGTLVTVSS

SEQ ID NO: 401 - protein, 5 aa, synthetic construct
  REGION 1..5: note = Synthetic Construct
TYAMN

SEQ ID NO: 402 - protein, 7 aa, synthetic construct
  REGION 1..7: note = Synthetic Construct
GFTFNTY

SEQ ID NO: 403 - protein, 10 aa, synthetic construct
  REGION 1..10: note = Synthetic Construct
GFTFNTYAMN

SEQ ID NO: 404 - protein, 8 aa, synthetic construct
  REGION 1..8: note = Synthetic Construct
RSKINNYA

SEQ ID NO: 405 - protein, 19 aa, synthetic construct
  REGION 1..19: note = Synthetic Construct
RIRSKINNYATYYAESVKG

SEQ ID NO: 406 - protein, 13 aa, synthetic construct
  REGION 1..13: note = Synthetic Construct
HETLRSGISWFAS

SEQ ID NO: 407 - protein, 7 aa, synthetic construct
  REGION 1..7: note = Synthetic Construct
GFTFSTY

SEQ ID NO: 408 - protein, 10 aa, synthetic construct
  REGION 1..10: note = Synthetic Construct
GFTFSTYAMN

SEQ ID NO: 409 - protein, 8 aa, synthetic construct
  REGION 1..8: note = Synthetic Construct
RSHINNYA

SEQ ID NO: 410 - protein, 19 aa, synthetic construct
  REGION 1..19: note = Synthetic Construct
RIRSHINNYATYYAESVKG

SEQ ID NO: 411 - protein, 8 aa, synthetic construct
  REGION 1..8: note = Synthetic Construct
RSKYNNYA

SEQ ID NO: 412 - protein, 19 aa, synthetic construct
  REGION 1..19: note = Synthetic Construct
RIRSKYNNYATYYAESVKG

SEQ ID NO: 413 - protein, 19 aa, synthetic construct
  REGION 1..19: note = Synthetic Construct
RERSKINNYATYYAESVKG

SEQ ID NO: 414 - protein, 19 aa, synthetic construct
  REGION 1..19: note = Synthetic Construct
RIRSKINNYKTYYAESVKG

SEQ ID NO: 415 - protein, 7 aa, synthetic construct
  REGION 1..7: note = Synthetic Construct
GFTFTDY

SEQ ID NO: 416 - protein, 10 aa, synthetic construct
  REGION 1..10: note = Synthetic Construct
GFTFTDYYMT

SEQ ID NO: 417 - protein, 8 aa, synthetic construct
  REGION 1..8: note = Synthetic Construct
RNRARGYT

SEQ ID NO: 418 - protein, 19 aa, synthetic construct
  REGION 1..19: note = Synthetic Construct
FIRNRARGYTSDHNASVKG

SEQ ID NO: 419 - protein, 7 aa, synthetic construct
  REGION 1..7: note = Synthetic Construct
GYTFTSY

SEQ ID NO: 420 - protein, 10 aa, synthetic construct
  REGION 1..10: note = Synthetic Construct
GYTFTSYWMH

SEQ ID NO: 421 - protein, 6 aa, synthetic construct
  REGION 1..6: note = Synthetic Construct
YSGGDT

SEQ ID NO: 422 - protein, 17 aa, synthetic construct
  REGION 1..17: note = Synthetic Construct
NIYSGGDTINYDEKFKN

SEQ ID NO: 423 - protein, 10 aa, synthetic construct
  REGION 1..10: note = Synthetic Construct
DATSRYFFDY

SEQ ID NO: 424 - protein, 5 aa, synthetic construct
  REGION 1..5: note = Synthetic Construct
TYYLH

SEQ ID NO: 425 - protein, 8 aa, synthetic construct
  REGION 1..8: note = Synthetic Construct
GYSFTTYY

SEQ ID NO: 426 - protein, 10 aa, synthetic construct
  REGION 1..10: note = Synthetic Construct
GYSFTTYYLH

SEQ ID NO: 427 - protein, 6 aa, synthetic construct
  REGION 1..6: note = Synthetic Construct
FPGSDN

SEQ ID NO: 428 - protein, 17 aa, synthetic construct
  REGION 1..17: note = Synthetic Construct
WIFPGSDNTKYNEKFKG

SEQ ID NO: 429 - protein, 8 aa, synthetic construct
  REGION 1..8: note = Synthetic Construct
NRDYYFDY

SEQ ID NO: 430 - protein, 17 aa, synthetic construct
  REGION 1..17: note = Synthetic Construct
TSSQSLFNSRSRKNYLA

SEQ ID NO: 431 - protein, 15 aa, synthetic construct
  REGION 1..15: note = Synthetic Construct
KSSQSLLNSRTRKNY

SEQ ID NO: 432 - protein, 8 aa, synthetic construct
  REGION 1..8: note = Synthetic Construct
TQSFILRT

SEQ ID NO: 433 - protein, 7 aa, synthetic construct
  REGION 1..7: note = Synthetic Construct
WASTRAS

SEQ ID NO: 434 - protein, 8 aa, synthetic construct
  REGION 1..8: note = Synthetic Construct
KQSFILRT

SEQ ID NO: 435 - protein, 14 aa, synthetic construct
  REGION 1..14: note = Synthetic Construct
RSSTGAVTTSNYAN

SEQ ID NO: 436 - protein, 7 aa, synthetic construct
  REGION 1..7: note = Synthetic Construct
GTNTRAP

SEQ ID NO: 437 - protein, 9 aa, synthetic construct
  REGION 1..9: note = Synthetic Construct
VLWYNNYWV

SEQ ID NO: 438 - protein, 9 aa, synthetic construct
  REGION 1..9: note = Synthetic Construct
ALWYSNHWV

SEQ ID NO: 439 - protein, 9 aa, synthetic construct
  REGION 1..9: note = Synthetic Construct
VLWYNNHWV

SEQ ID NO: 440 - protein, 14 aa, synthetic construct
  REGION 1..14: note = Synthetic Construct
RASTGAVTTSNYAN

SEQ ID NO: 441 - protein, 14 aa, synthetic construct
  REGION 1..14: note = Synthetic Construct
RTSTGAVTTSNYAN

SEQ ID NO: 442 - protein, 117 aa, synthetic construct
  REGION 1..117: note = Synthetic Construct
EVQLQQSGAELVRPGALVKLSCKGSGFNIKDYYIHWVKQRPEQGLEWIGWIDPENGNNKYDPKFQGKASITADTSSNIAYLQLSSLTSEDTAVYYCARNDNYAFDYWGQGTTVTVSS

SEQ ID NO: 443 - protein, 112 aa, synthetic construct
  REGION 1..112: note = Synthetic Construct
DIVVSQSPSSLAVSAGEKVIMSCKSSQSLLNSRTRKNYLAWYQLKPGQSPKLLIYSASTRESGVPDRFTGSGSGTDFTLTISSVQTEDLAVYYCMQSFTLRTFGGGTKLEIK

SEQ ID NO: 444 - protein, 121 aa, synthetic construct; identical to SEQ ID NO: 320
  REGION 1..121: note = Synthetic Construct

SEQ ID NO: 445 - protein, 112 aa, synthetic construct
  REGION 1..112: note = Synthetic Construct
DIVMTQSPDSLAVSLGERATINCTSSQSLFNSRSRKNYLAWYQQKPGQPPKLLISWASTRESGVPDRFSGSGSGTDFTLTISSLQAEDVAVYYCQQSYDTFTFGSGTKLEIK

SEQ ID NO: 446 - protein, 5 aa, synthetic construct
  REGION 1..5: note = Synthetic Construct
DYYIH

SEQ ID NO: 447 - protein, 7 aa, synthetic construct
  REGION 1..7: note = Synthetic Construct
GFNIKDY

SEQ ID NO: 448 - protein, 10 aa, synthetic construct
  REGION 1..10: note = Synthetic Construct
GFNIKDYYIH

SEQ ID NO: 449 - protein, 6 aa, synthetic construct
  REGION 1..6: note = Synthetic Construct
DPENGN

SEQ ID NO: 450 - protein, 17 aa, synthetic construct
  REGION 1..17: note = Synthetic Construct
WIDPENGNNKYDPKFQG

SEQ ID NO: 451 - protein, 8 aa, synthetic construct
  REGION 1..8: note = Synthetic Construct
NDNYAFDY

SEQ ID NO: 452 - protein, 7 aa, synthetic construct
  REGION 1..7: note = Synthetic Construct
SASTRES

SEQ ID NO: 453 - protein, 8 aa, synthetic construct
  REGION 1..8: note = Synthetic Construct
MQSFTLRT

SEQ ID NO: 454 - protein, 4 aa, synthetic construct
  REGION 1..4: note = Synthetic Construct
LLQG

SEQ ID NO: 455 - protein, 6 aa, synthetic construct
  REGION 1..6: note = Synthetic Construct
LSLSQG

SEQ ID NO: 456 - protein, 8 aa, synthetic construct
  REGION 1..8: note = Synthetic Construct
GGGLLQGG

SEQ ID NO: 457 - protein, 5 aa, synthetic construct
  REGION 1..5: note = Synthetic Construct
GLLQG

SEQ ID NO: 458 - protein, 10 aa, synthetic construct
  REGION 1..10: note = Synthetic Construct
GSPLAQSHGG

SEQ ID NO: 459 - protein, 7 aa, synthetic construct
  REGION 1..7: note = Synthetic Construct
GLLQGGG

SEQ ID NO: 460 - protein, 6 aa, synthetic construct
  REGION 1..6: note = Synthetic Construct
GLLQGG

SEQ ID NO: 461 - protein, 4 aa, synthetic construct
  REGION 1..4: note = Synthetic Construct
GLLQ

SEQ ID NO: 462 - protein, 8 aa, synthetic construct
  REGION 1..8: note = Synthetic Construct
LLQLLQGA

SEQ ID NO: 463 - protein, 5 aa, synthetic construct
  REGION 1..5: note = Synthetic Construct
LLQGA

SEQ ID NO: 464 - protein, 7 aa, synthetic construct
  REGION 1..7: note = Synthetic Construct
LLQYQGA

SEQ ID NO: 465 - protein, 6 aa, synthetic construct
  REGION 1..6: note = Synthetic Construct
LLQGSG

SEQ ID NO: 466 - protein, 6 aa, synthetic construct
  REGION 1..6: note = Synthetic Construct
LLQYQG

SEQ ID NO: 467 - protein, 7 aa, synthetic construct
  REGION 1..7: note = Synthetic Construct
LLQLLQG

SEQ ID NO: 468 - protein, 5 aa, synthetic construct
  REGION 1..5: note = Synthetic Construct
SLLQG

SEQ ID NO: 469 - protein, 5 aa, synthetic construct
  REGION 1..5: note = Synthetic Construct
LLQLQ

SEQ ID NO: 470 - protein, 6 aa, synthetic construct
  REGION 1..6: note = Synthetic Construct
LLQLLQ

SEQ ID NO: 471 - protein, 5 aa, synthetic construct
  REGION 1..5: note = Synthetic Construct
LLQGR

SEQ ID NO: 472 - protein, 6 aa, synthetic construct
  REGION 1..6: note = Synthetic Construct
LLQGPP

SEQ ID NO: 473 - protein, 6 aa, synthetic construct
  REGION 1..6: note = Synthetic Construct
LLQGPA

SEQ ID NO: 474 - protein, 8 aa, synthetic construct
  REGION 1..8: note = Synthetic Construct
GGLLQGPP

SEQ ID NO: 475 - protein, 7 aa, synthetic construct
  REGION 1..7: note = Synthetic Construct
GGLLQGA

SEQ ID NO: 476 - protein, 7 aa, synthetic construct
  REGION 1..7: note = Synthetic Construct
LLQGPGK

SEQ ID NO: 477 - protein, 6 aa, synthetic construct
  REGION 1..6: note = Synthetic Construct
LLQGPG

SEQ ID NO: 478 - protein, 5 aa, synthetic construct
  REGION 1..5: note = Synthetic Construct
LLQGP

SEQ ID NO: 479 - protein, 4 aa, synthetic construct
  REGION 1..4: note = Synthetic Construct
LLQP

SEQ ID NO: 480 - protein, 6 aa, synthetic construct
  REGION 1..6: note = Synthetic Construct
LLQPGK

SEQ ID NO: 481 - protein, 7 aa, synthetic construct
  REGION 1..7: note = Synthetic Construct
LLQAPGK

SEQ ID NO: 482 - protein, 7 aa, synthetic construct
  REGION 1..7: note = Synthetic Construct
LLQGAPG

SEQ ID NO: 483 - protein, 6 aa, synthetic construct
  REGION 1..6: note = Synthetic Construct
LLQGAP

SEQ ID NO: 484 - protein, 6 aa, synthetic construct
  REGION 1..6: note = Synthetic Construct
LLQLQG

SEQ ID NO: 485 - DNA, 255 bp, synthetic construct
  misc_feature 1..255: note = Synthetic Construct
  source 1..255: mol_type = other DNA
gagatcgtgctgactcagtcccctggaaccctgtccctgtcacctggcgaaagagctaccttgtcctgtcgcgcatcacaatccgtgtcgtcgagctatctcgcgtggtaccagcagaagcccggacaggccccaaggctgcttatgtacgacgcctccatccgggccactggtatccccgaccgcttctcgggctccggaagcggcaccgacttcaccctgactatttcccggctcgaaccggaggatttcgcc

SEQ ID NO: 486 - DNA, 255 bp, synthetic construct
  misc_feature 1..255: note = Synthetic Construct
  source 1..255: mol_type = other DNA
gaagtccaactcctcgaatccggtggcggccttgtccagcctggaggttccttgcgcctgtcatgtgccgccagcggattcaccttctcgtcctacccgatgtcgtgggtccgccaggctccgggaaagggcctggaatgggtgtcagccatcggaggatcggggggctccctgccctacgccgatatcgtgaagggaaggttcaccattagccgggacaactccaagaacactctgtacctccaaatgaacagc

SEQ ID NO: 487 - DNA, 255 bp, synthetic construct
  misc_feature 1..255: note = Synthetic Construct
  source 1..255: mol_type = other DNA
gagatcgtgctgacacagagccctggcaccctgagcctgtctccaggcgaaagagccaccctgtcctgcagagccagccagagcgtgtccagcagctacctggcctggtatcagcagaagcccggccaggctccccggctgctgatctatggcgcctcttctagagccaccggcatccccgatagattcagcggctctggcagcggcaccgacttcaccctgaccatcagcagactggaacccgaggacttcgcc

SEQ ID NO: 488 - DNA, 255 bp, synthetic construct
  misc_feature 1..255: note = Synthetic Construct
  source 1..255: mol_type = other DNA
gaagtgcagctgctggaatctggcggaggactggtgcagcctggcggctctctgagactgtcttgtgccgccagcggcttcaccttcggcagctacgctatgacctgggtgcgccaggcccctggcaaaggactggaatgggtgtccgccatctctggcagcggcggcaataccttctacgccgagagcgtgaagggccggttcaccatcagccgggacaacagcaagaacaccctgtacctgcagatgaacagc

SEQ ID NO: 489 - DNA, 255 bp, synthetic construct
  misc_feature 1..255: note = Synthetic Construct
  source 1..255: mol_type = other DNA
gagatcgtgctgacacagagccctggcaccctgagcctgtctcctggtgaaagagctactttgtcttgtagagcttctcaatccgtttccgcgtattatttggcttggtatcaacaaaaaccaggtcaagctccaagattattgatgtacgatgcttctattagagccaccggtattccagatagattttctggttctggttccggtactgatttcactttgactatctctagattggaaccagaagatttcgct

SEQ ID NO: 490 - DNA, 255 bp, synthetic construct
  misc_feature 1..255: note = Synthetic Construct
  source 1..255: mol_type = other DNA
gaagttcaattattggaatctggtggaggactggtgcagcctggcggctctctgagactgtcttgtgccgccagcggcttcaccttcagcagctacgccatgaactgggtgcgccaggcccctggtaaaggtttggaatgggtttctgctattactgcgtctggtggttctacttactatgccgatgtggttaagggtagattcaccatttctagagacaactctaagaacaccttgtacttgcaaatgaactcc

SEQ ID NO: 491 - DNA, 255 bp, synthetic construct
  misc_feature 1..255: note = Synthetic Construct
  source 1..255: mol_type = other DNA
gagatcgtgctgacacagagccctggcaccctgagcctgtctcctggtgaaagagctactttgtcttgtagagcttctcaatccgtttccgatctgtatttggcttggtatcaacaaaaaccaggtcaagctccaagattattgatgtacgatgcttctattagagccaccggtattccagatagattttctggttctggttccggtactgatttcactttgactatctctagattggaaccagaagatttcgct

SEQ ID NO: 492 - DNA, 255 bp, synthetic construct
  misc_feature 1..255: note = Synthetic Construct
  source 1..255: mol_type = other DNA
gaagttcaattattggaatctggtggaggactggtgcagcctggcggctctctgagactgtcttgtgccgccagcggcttcaccttcagcagctacgccatgaactgggtgcgccaggcccctggtaaaggtttggaatgggtttctgctatttctgattttggtggttctacttactatgccgatatcgttaagggtagattcaccatttctagagacaactctaagaacaccttgtacttgcaaatgaactcc

SEQ ID NO: 493 - protein, 255 aa, Homo sapiens
ASTKGPSVFPLAPCSRSTSESTAALGCLVKDYFPEPVTVSWNSGALTSGVHTFPAVLQSSGLYSLSSVVTVPSSNFGTQTYTCNVDHKPSNTKVDKTVERKCCVECPPCPAPPVAGPSVFLFPPKPKDTLMISRTPEVTCVVVDVSHEDPEVQFNWYVDGVEVHNAKTKPREEQFNSTFRVVSVLTVVHQDWLNGKEYKCKVSNKGLPAPIEKTISKTKGQPREPQVYTLPPSREEMTKNQVSLTCLVKGFYPSD

SEQ ID NO: 494 - protein, 255 aa, Homo sapiens
ASTKGPSVFPLAPSSKSTSGGTAALGCLVKDYFPEPVTVSWNSGALTSGVHTFPAVLQSSGLYSLSSVVTVPSSSLGTQTYICNVNHKPSNTKVDKKVEPKSCDKTHTCPPCPAPELLGGPSVFLFPPKPKDTLMISRTPEVTCVVVDVSHEDPEVKFNWYVDGVEVHNAKTKPREEQYNSTYRVVSVLTVLHQDWLNGKEYKCKVSNKALPAPIEKTISKAKGQPREPQVYTLPPSREEMTKNQVSLTCLVKGF

SEQ ID NO: 495 - protein, 255 aa, Homo sapiens; identical to SEQ ID NO: 494

SEQ ID NO: 496 - protein, 255 aa, synthetic construct
  REGION 1..255: note = Synthetic Construct
ASTKGPSVFPLAPCSRSTSESTAALGCLVKDYFPEPVTVSWNSGALTSGVHTFPAVLQSSGLYSLSSVVTVPSSNFGTQTYTCNVDHKPSNTKVDKTVERKCRVRCPRCPAPPVAGPSVFLFPPKPKDTLMISRTPEVTCVVVAVSHEDPEVQFNWYVDGVEVHNAKTKPREEQFNSTFRVVSVLTVVHQDWLNGKEYKCKVSNKGLPSSIEKTISKTKGQPREPQVYTLPPSREEMTKNQVSLTCLVKGFYPSD

SEQ ID NO: 497 - protein, 255 aa, synthetic construct
  REGION 1..255: note = Synthetic Construct
ASTKGPSVFPLAPCSRSTSESTAALGCLVKDYFPEPVTVSWNSGALTSGVHTFPAVLQSSGLYSLSSVVTVPSSNFGTQTYTCNVDHKPSNTKVDKTVERKCEVECPECPAPPVAGPSVFLFPPKPKDTLMISRTPEVTCVVVAVSHEDPEVQFNWYVDGVEVHNAKTKPREEQFNSTFRVVSVLTVVHQDWLNGKEYKCKVSNKGLPSSIEKTISKTKGQPREPQVYTLPPSREEMTKNQVSLTCEVKGFYPSD

SEQ ID NO: 498 - protein, 15 aa, synthetic construct
  REGION 1..15: note = Synthetic Construct
GGGGSGGGGSGGGGS

SEQ ID NO: 499 - protein, 10 aa, synthetic construct
  REGION 1..10: note = Synthetic Construct
QHYGSPPLFT

SEQ ID NO: 500 - protein, 12 aa, synthetic construct
  REGION 1..12: note = Synthetic Construct
RASQNVSSSYLA

SEQ ID NO: 501 - protein, 7 aa, synthetic construct
  REGION 1..7: note = Synthetic Construct
GASYRAT

SEQ ID NO: 502 - protein, 198 aa, Homo sapiens
MQSGTRWRVLGLCLLSIGVWGQDGNEEMGSITQTPYQVSISGTTVILTCSQHLGSEAQWQHNGKNKEDSGDRLFLPEFSEMEQSGYYVCYPRGSNPEDASHHLYLKARVCENCMEMDVMAVATIVIVDICITLGLLLLVYYWSKNRKAKAKPVTRGAGAGGRQRGQNKERPPPVPNPDYEPIRKGQQDLYSGLNQRRI